European Patent Application EP 4 706 769 A2, published March 11, 2026. Title: ANTI-CD47 ANTIBODIES AND METHODS OF USE THEREOF. Applicant: Novimmune SA. The sequence listing filed with the application follows.

SEQUENCE LISTING (287 sequences)

SEQ ID NO: 1 - DNA, 1338 bp, synthetic construct
  misc_feature 1..1338: note = common heavy chain
  source 1..1338: mol_type = other DNA
gaggtgcagctgttggagtctgggggaggcttggtacagcctggggggtccctgagactctcctgtgcagcctctggattcacctttagcagctatgccatgagctgggtccgccaggctccagggaaggggctggagtgggtctcagctattagtggtagtggtggtagcacatactacgcagactccgtgaagggccggttcaccatctccagagacaattccaagaacacgctgtatctgcaaatgaacagcctgagagccgaggacacggccgtatattactgtgcgaaaagttatggtgcttttgactactggggccagggaaccctggtcacagtctcgagcgcctccaccaagggcccatcggtcttccccctggcaccctcctccaagagcacctctgggggcacagcggccctgggctgcctggtcaaggactacttccccgaaccggtgacagtctcgtggaactcaggagccctgaccagcggcgtgcacaccttcccggctgtcctacagtcctcaggactctactccctcagcagcgtggtgactgtgccctccagcagcttgggcacccagacctacatctgcaacgtgaatcacaagcccagcaacaccaaggtggacaagagagttgagcccaaatcttgtgacaaaactcacacatgcccaccgtgcccagcacctgaactcctggggggaccgtcagtcttcctcttccccccaaaacccaaggacaccctcatgatctcccggacccctgaggtcacatgcgtggtggtggacgtgagccacgaagaccctgaggtcaagttcaactggtacgtggacggcgtggaggtgcataatgccaagacaaagccgcgggaggagcagtacaacagcacgtaccgtgtggtcagcgtcctcaccgtcctgcaccaggactggctgaatggcaaggagtacaagtgcaaggtctccaacaaagccctcccagcccccatcgagaaaaccatctccaaagccaaagggcagccccgagaaccacaggtgtataccctgcccccatctcgggaggagatgaccaagaaccaggtcagcctgacttgcctggtcaaaggcttctatcccagcgacatcgccgtggagtgggagagcaacgggcagccggagaacaactacaagaccacgcctcccgtgctggactccgacggctccttcttcctctatagcaagctcaccgtggacaagtccaggtggcagcaggggaacgtcttctcatgctccgtgatgcatgaggctctgcacaaccactacacgcagaagagcctctccctgtctccgggttaa

SEQ ID NO: 2 - protein, 445 aa, synthetic construct
  REGION 1..445: note = common heavy chain
EVQLLESGGGLVQPGGSLRLSCAASGFTFSSYAMSWVRQAPGKGLEWVSAISGSGGSTYYADSVKGRFTISRDNSKNTLYLQMNSLRAEDTAVYYCAKSYGAFDYWGQGTLVTVSSASTKGPSVFPLAPSSKSTSGGTAALGCLVKDYFPEPVTVSWNSGALTSGVHTFPAVLQSSGLYSLSSVVTVPSSSLGTQTYICNVNHKPSNTKVDKRVEPKSCDKTHTCPPCPAPELLGGPSVFLFPPKPKDTLMISRTPEVTCVVVDVSHEDPEVKFNWYVDGVEVHNAKTKPREEQYNSTYRVVSVLTVLHQDWLNGKEYKCKVSNKALPAPIEKTISKAKGQPREPQVYTLPPSREEMTKNQVSLTCLVKGFYPSDIAVEWESNGQPENNYKTTPPVLDSDGSFFLYSKLTVDKSRWQQGNVFSCSVMHEALHNHYTQKSLSLSPG

SEQ ID NO: 3 - DNA, 648 bp, synthetic construct
  misc_feature 1..648: note = anti-CD47 5A3 kappa light chain
  source 1..648: mol_type = other DNA
gacatccagatgacccagtctccatcctccctgtctgcatctgtaggagacagagtcaccatcacttgccaggcgagtcaggacattaataagtatttaaattggtatcagcagaaaccagggaaagcccctaagctcctgatctacggtgcatccaggttggaaacaggggtcccatcaaggttcagtggaagtggatctgggacagattttactttcaccatcagcagcctgcagcctgaagatattgcaacatattactgtcagcagaagcacccccgggggccgaggaccttcggccaagggaccaaggtggaaatcaaacgtacggtggctgcaccatctgtcttcatcttcccgccatctgatgagcagttgaaatctggaactgcctctgttgtgtgcctgctgaataacttctatcccagagaggccaaagtacagtggaaggtggataacgccctccaatcgggtaactcccaggagagtgtcacagagcaggacagcaaggacagcacctacagcctcagcagcaccctgacgctgagcaaagcagactacgagaaacacaaagtctacgcctgcgaagtcacccatcagggcctgagctcgcccgtcacaaagagcttcaacaggggagagtgttaa

SEQ ID NO: 4 - protein, 215 aa, synthetic construct
  REGION 1..215: note = anti-CD47 5A3 kappa light chain
DIQMTQSPSSLSASVGDRVTITCQASQDINKYLNWYQQKPGKAPKLLIYGASRLETGVPSRFSGSGSGTDFTFTISSLQPEDIATYYCQQKHPRGPRTFGQGTKVEIKRTVAAPSVFIFPPSDEQLKSGTASVVCLLNNFYPREAKVQWKVDNALQSGNSQESVTEQDSKDSTYSLSSTLTLSKADYEKHKVYACEVTHQGLSSPVTKSFNRGEC

SEQ ID NO: 5 - DNA, 648 bp, synthetic construct
  misc_feature 1..648: note = anti-CD47 5A3-M4 kappa light chain
  source 1..648: mol_type = other DNA
gacatccagatgacccagtctccatcctccctgtctgcatctgtaggagacagagtcaccatcacttgccaggcgagtcaggacattaataagtatttaaattggtatcagcagaaaccagggaaagcccctaagctcctgatctacggtgcatccaggttggaaacaggggtcccatcaaggttcagtggaagtggatctgggacagattttactttcaccatcagcagcctgcagcctgaagatattgcaacatattactgtcagcagaagcacccccggaacccgaggaccttcggccaagggaccaaggtggaaatcaaacgtacggtggctgcaccatctgtcttcatcttcccgccatctgatgagcagttgaaatctggaactgcctctgttgtgtgcctgctgaataacttctatcccagagaggccaaagtacagtggaaggtggataacgccctccaatcgggtaactcccaggagagtgtcacagagcaggacagcaaggacagcacctacagcctcagcagcaccctgacgctgagcaaagcagactacgagaaacacaaagtctacgcctgcgaagtcacccatcagggcctgagctcgcccgtcacaaagagcttcaacaggggagagtgttaa

SEQ ID NO: 6 - protein, 215 aa, synthetic construct
  REGION 1..215: note = anti-CD47 5A3-M4 kappa light chain
DIQMTQSPSSLSASVGDRVTITCQASQDINKYLNWYQQKPGKAPKLLIYGASRLETGVPSRFSGSGSGTDFTFTISSLQPEDIATYYCQQKHPRNPRTFGQGTKVEIKRTVAAPSVFIFPPSDEQLKSGTASVVCLLNNFYPREAKVQWKVDNALQSGNSQESVTEQDSKDSTYSLSSTLTLSKADYEKHKVYACEVTHQGLSSPVTKSFNRGEC

SEQ ID NO: 7 - DNA, 648 bp, synthetic construct
  misc_feature 1..648: note = anti-CD47 5A3-M3 kappa light chain
  source 1..648: mol_type = other DNA
gacatccagatgacccagtctccatcctccctgtctgcatctgtaggagacagagtcaccatcacttgccaggcgagtcagtccattagtagttatttaaattggtatcagcagaaaccagggaaagcccctaagctcctgatctacgctgcatcctcgttggaaacaggggtcccatcaaggttcagtggaagtggatctgggacagattttactttcaccatcagcagcctgcagcctgaagatattgcaacatattactgtcagcagaagcacccccgggggccgaggaccttcggccaagggaccaaggtggaaatcaaacgtacggtggctgcaccatctgtcttcatcttcccgccatctgatgagcagttgaaatctggaactgcctctgttgtgtgcctgctgaataacttctatcccagagaggccaaagtacagtggaaggtggataacgccctccaatcgggtaactcccaggagagtgtcacagagcaggacagcaaggacagcacctacagcctcagcagcaccctgacgctgagcaaagcagactacgagaaacacaaagtctacgcctgcgaagtcacccatcagggcctgagctcgcccgtcacaaagagcttcaacaggggagagtgttaa

SEQ ID NO: 8 - protein, 215 aa, synthetic construct
  REGION 1..215: note = anti-CD47 5A3-M3 kappa light chain
DIQMTQSPSSLSASVGDRVTITCQASQSISSYLNWYQQKPGKAPKLLIYAASSLETGVPSRFSGSGSGTDFTFTISSLQPEDIATYYCQQKHPRGPRTFGQGTKVEIKRTVAAPSVFIFPPSDEQLKSGTASVVCLLNNFYPREAKVQWKVDNALQSGNSQESVTEQDSKDSTYSLSSTLTLSKADYEKHKVYACEVTHQGLSSPVTKSFNRGEC

SEQ ID NO: 9 - DNA, 648 bp, synthetic construct
  misc_feature 1..648: note = anti-CD47 5A3-M5 kappa light chain
  source 1..648: mol_type = other DNA
gacatccagatgacccagtctccatcctccctgtctgcatctgtaggagacagagtcaccatcacttgccaggcgagtcaggacattaataagtatttaaattggtatcagcagaaaccagggaaagcccctaagctcctgatctacggtgcatccaggttggaaacaggggtcccatcaaggttcagtggaagtggatctgggacagattttactttcaccatcagcagcctgcagcctgaagatattgcaacatattactgtcagcagaagcacccccggtacccgaggaccttcggccaagggaccaaggtggaaatcaaacgtacggtggctgcaccatctgtcttcatcttcccgccatctgatgagcagttgaaatctggaactgcctctgttgtgtgcctgctgaataacttctatcccagagaggccaaagtacagtggaaggtggataacgccctccaatcgggtaactcccaggagagtgtcacagagcaggacagcaaggacagcacctacagcctcagcagcaccctgacgctgagcaaagcagactacgagaaacacaaagtctacgcctgcgaagtcacccatcagggcctgagctcgcccgtcacaaagagcttcaacaggggagagtgttaa

SEQ ID NO: 10 - protein, 215 aa, synthetic construct
  REGION 1..215: note = anti-CD47 5A3-M5 kappa light chain
DIQMTQSPSSLSASVGDRVTITCQASQDINKYLNWYQQKPGKAPKLLIYGASRLETGVPSRFSGSGSGTDFTFTISSLQPEDIATYYCQQKHPRYPRTFGQGTKVEIKRTVAAPSVFIFPPSDEQLKSGTASVVCLLNNFYPREAKVQWKVDNALQSGNSQESVTEQDSKDSTYSLSSTLTLSKADYEKHKVYACEVTHQGLSSPVTKSFNRGEC

SEQ ID NO: 11 - DNA, 648 bp, synthetic construct
  misc_feature 1..648: note = anti-CD47 Ke8 kappa light chain
  source 1..648: mol_type = other DNA
gacatccagatgacccagtctccatcctccctgtctgcatctgtaggagacagagtcaccatcacttgccgggcaagtcagagcattagcagctatttaaattggtatcagcagaaaccagggaaagcccctaagctcctgatctatgctgcatccagtttgcaaagtggggtcccatcaaggttcagtggcagtggatctgggacagatttcactctcaccatcagcagtctgcaacctgaagattttgcaacttactactgtcagcagttccacaagcggcggccgcagaccttcggccaagggaccaaggtggaaatcaaacgtacggtggctgcaccatctgtcttcatcttcccgccatctgatgagcagttgaaatctggaactgcctctgttgtgtgcctgctgaataacttctatcccagagaggccaaagtacagtggaaggtggataacgccctccaatcgggtaactcccaggagagtgtcacagagcaggacagcaaggacagcacctacagcctcagcagcaccctgacgctgagcaaagcagactacgagaaacacaaagtctacgcctgcgaagtcacccatcagggcctgagctcgcccgtcacaaagagcttcaacaggggagagtgttaa

SEQ ID NO: 12 - protein, 215 aa, synthetic construct
  REGION 1..215: note = anti-CD47 Ke8 kappa light chain
DIQMTQSPSSLSASVGDRVTITCRASQSISSYLNWYQQKPGKAPKLLIYAASSLQSGVPSRFSGSGSGTDFTLTISSLQPEDFATYYCQQFHKRRPQTFGQGTKVEIKRTVAAPSVFIFPPSDEQLKSGTASVVCLLNNFYPREAKVQWKVDNALQSGNSQESVTEQDSKDSTYSLSSTLTLSKADYEKHKVYACEVTHQGLSSPVTKSFNRGEC

SEQ ID NO: 13 - DNA, 648 bp, synthetic construct
  misc_feature 1..648: note = anti-CD47 Ke8H5 kappa light chain
  source 1..648: mol_type = other DNA
gacatccagatgacccagtctccatcctccctgtctgcatctgtaggagacagagtcaccatcacttgccgggcaagtcagagcattgcgaggtatttaaattggtatcagcagaaaccagggaaagcccctaagctcctgatctatgctgcatccagtttgcaaagtggggtcccatcaaggttcagtggcagtggatctgggacagatttcactctcaccatcagcagtctgcaacctgaagattttgcaacttactactgtcagcagttccataagcgtgcgccgcagaccttcggccaagggaccaaggtggaaatcaaacgtacggtggctgcaccatctgtcttcatcttcccgccatctgatgagcagttgaaatctggaactgcctctgttgtgtgcctgctgaataacttctatcccagagaggccaaagtacagtggaaggtggataacgccctccaatcgggtaactcccaggagagtgtcacagagcaggacagcaaggacagcacctacagcctcagcagcaccctgacgctgagcaaagcagactacgagaaacacaaagtctacgcctgcgaagtcacccatcagggcctgagctcgcccgtcacaaagagcttcaacaggggagagtgttaa

SEQ ID NO: 14 - protein, 215 aa, synthetic construct
  REGION 1..215: note = anti-CD47 Ke8H5 kappa light chain
DIQMTQSPSSLSASVGDRVTITCRASQSIARYLNWYQQKPGKAPKLLIYAASSLQSGVPSRFSGSGSGTDFTLTISSLQPEDFATYYCQQFHKRAPQTFGQGTKVEIKRTVAAPSVFIFPPSDEQLKSGTASVVCLLNNFYPREAKVQWKVDNALQSGNSQESVTEQDSKDSTYSLSSTLTLSKADYEKHKVYACEVTHQGLSSPVTKSFNRGEC

SEQ ID NO: 15 - DNA, 648 bp, synthetic construct
  misc_feature 1..648: note = anti-CD47 Ke8B2 kappa light chain
  source 1..648: mol_type = other DNA
gacatccagatgacccagtctccatcctccctgtctgcatctgtaggagacagagtcaccatcacttgccgggcaagtcagagcattggtaagtatttaaattggtatcagcagaaaccagggaaagcccctaagctcctgatctatgcggcatccaggttgcaaagtggggtcccatcaaggttcagtggcagtggatctgggacagatttcactctcaccatcagcagtctgcaacctgaagattttgcaacttactactgtcagcagaagcacccgcgtgccccgcggaccttcggccaagggaccaaggtggaaatcaaacgtacggtggctgcaccatctgtcttcatcttcccgccatctgatgagcagttgaaatctggaactgcctctgttgtgtgcctgctgaataacttctatcccagagaggccaaagtacagtggaaggtggataacgccctccaatcgggtaactcccaggagagtgtcacagagcaggacagcaaggacagcacctacagcctcagcagcaccctgacgctgagcaaagcagactacgagaaacacaaagtctacgcctgcgaagtcacccatcagggcctgagctcgcccgtcacaaagagcttcaacaggggagagtgttaa

SEQ ID NO: 16 - protein, 215 aa, synthetic construct
  REGION 1..215: note = anti-CD47 Ke8B2 kappa light chain
DIQMTQSPSSLSASVGDRVTITCRASQSIGKYLNWYQQKPGKAPKLLIYAASRLQSGVPSRFSGSGSGTDFTLTISSLQPEDFATYYCQQKHPRAPRTFGQGTKVEIKRTVAAPSVFIFPPSDEQLKSGTASVVCLLNNFYPREAKVQWKVDNALQSGNSQESVTEQDSKDSTYSLSSTLTLSKADYEKHKVYACEVTHQGLSSPVTKSFNRGEC

SEQ ID NO: 17 - DNA, 648 bp, synthetic construct
  misc_feature 1..648: note = anti-CD47 Ke8A2 kappa light chain
  source 1..648: mol_type = other DNA
gacatccagatgacccagtctccatcctccctgtctgcatctgtaggagacagagtcaccatcacttgccgggcaagtcagagcattgataggtatttaaattggtatcagcagaaaccagggaaagcccctaagctcctgatctatgctgcatccagtttgcaaagtggggtcccatcaaggttcagtggcagtggatctgggacagatttcactctcaccatcagcagtctgcaacctgaagattttgcaacttactactgtcagcagaagcatccccgtgggccgaggaccttcggccaagggaccaaggtggaaatcaaacgtacggtggctgcaccatctgtcttcatcttcccgccatctgatgagcagttgaaatctggaactgcctctgttgtgtgcctgctgaataacttctatcccagagaggccaaagtacagtggaaggtggataacgccctccaatcgggtaactcccaggagagtgtcacagagcaggacagcaaggacagcacctacagcctcagcagcaccctgacgctgagcaaagcagactacgagaaacacaaagtctacgcctgcgaagtcacccatcagggcctgagctcgcccgtcacaaagagcttcaacaggggagagtgttaa

SEQ ID NO: 18 - protein, 215 aa, synthetic construct
  REGION 1..215: note = anti-CD47 Ke8A2 kappa light chain
DIQMTQSPSSLSASVGDRVTITCRASQSIDRYLNWYQQKPGKAPKLLIYAASSLQSGVPSRFSGSGSGTDFTLTISSLQPEDFATYYCQQKHPRGPRTFGQGTKVEIKRTVAAPSVFIFPPSDEQLKSGTASVVCLLNNFYPREAKVQWKVDNALQSGNSQESVTEQDSKDSTYSLSSTLTLSKADYEKHKVYACEVTHQGLSSPVTKSFNRGEC

SEQ ID NO: 19 - DNA, 648 bp, synthetic construct
  misc_feature 1..648: note = anti-CD47 Ke8E8 kappa light chain
  source 1..648: mol_type = other DNA
gacatccagatgacccagtctccatcctccctgtctgcatctgtaggagacagagtcaccatcacttgccaggcgagtcaggacattaataagtatttaaattggtatcagcagaaaccagggaaagcccctaagctcctgatctatgctgcatccagtttgcaaagtggggtcccatcaaggttcagtggcagtggatctgggacagatttcactctcaccatcagcagtctgcaacctgaagattttgcaacttactactgtcagcagaagcatccccgtggcccgcggaccttcggccaagggaccaaggtggaaatcaaacgtacggtggctgcaccatctgtcttcatcttcccgccatctgatgagcagttgaaatctggaactgcctctgttgtgtgcctgctgaataacttctatcccagagaggccaaagtacagtggaaggtggataacgccctccaatcgggtaactcccaggagagtgtcacagagcaggacagcaaggacagcacctacagcctcagcagcaccctgacgctgagcaaagcagactacgagaaacacaaagtctacgcctgcgaagtcacccatcagggcctgagctcgcccgtcacaaagagcttcaacaggggagagtgttaa

SEQ ID NO: 20 - protein, 215 aa, synthetic construct
  REGION 1..215: note = anti-CD47 Ke8E8 kappa light chain
DIQMTQSPSSLSASVGDRVTITCQASQDINKYLNWYQQKPGKAPKLLIYAASSLQSGVPSRFSGSGSGTDFTLTISSLQPEDFATYYCQQKHPRGPRTFGQGTKVEIKRTVAAPSVFIFPPSDEQLKSGTASVVCLLNNFYPREAKVQWKVDNALQSGNSQESVTEQDSKDSTYSLSSTLTLSKADYEKHKVYACEVTHQGLSSPVTKSFNRGEC

SEQ ID NO: 21 - DNA, 648 bp, synthetic construct
  misc_feature 1..648: note = anti-CD47 Ke8H3 kappa light chain
  source 1..648: mol_type = other DNA
gacatccagatgacccagtctccatcctccctgtctgcatctgtaggagacagagtcaccatcacttgccgggcaagtcagagcattaataggtatttaaattggtatcagcagaaaccagggaaagcccctaagctcctgatctatgctgcatccaggttgcaaagtggggtcccatcaaggttcagtggcagtggatctgggacagatttcactctcaccatcagcagtctgcaacctgaagattttgcaacttactactgtcagcagaagcatccgcgtgggccgaggaccttcggccaagggaccaaggtggaaatcaaacgtacggtggctgcaccatctgtcttcatcttcccgccatctgatgagcagttgaaatctggaactgcctctgttgtgtgcctgctgaataacttctatcccagagaggccaaagtacagtggaaggtggataacgccctccaatcgggtaactcccaggagagtgtcacagagcaggacagcaaggacagcacctacagcctcagcagcaccctgacgctgagcaaagcagactacgagaaacacaaagtctacgcctgcgaagtcacccatcagggcctgagctcgcccgtcacaaagagcttcaacaggggagagtgttaa

SEQ ID NO: 22 - protein, 215 aa, synthetic construct
  REGION 1..215: note = anti-CD47 Ke8H3 kappa light chain
DIQMTQSPSSLSASVGDRVTITCRASQSINRYLNWYQQKPGKAPKLLIYAASRLQSGVPSRFSGSGSGTDFTLTISSLQPEDFATYYCQQKHPRGPRTFGQGTKVEIKRTVAAPSVFIFPPSDEQLKSGTASVVCLLNNFYPREAKVQWKVDNALQSGNSQESVTEQDSKDSTYSLSSTLTLSKADYEKHKVYACEVTHQGLSSPVTKSFNRGEC

SEQ ID NO: 23 - DNA, 648 bp, synthetic construct
  misc_feature 1..648: note = anti-CD47 Ke8G6 kappa light chain
  source 1..648: mol_type = other DNA
gacatccagatgacccagtctccatcctccctgtctgcatctgtaggagacagagtcaccatcacttgccgggcaagtcagagcattggtaggtatttaaattggtatcagcagaaaccagggaaagcccctaagctcctgatctatgctgcatccagtttgcaaagtggggtcccatcaaggttcagtggcagtggatctgggacagatttcactctcaccatcagcagtctgcaacctgaagattttgcaacttactactgtcagcagatgcatccgcgtgcgccgaagaccttcggccaagggaccaaggtggaaatcaaacgtacggtggctgcaccatctgtcttcatcttcccgccatctgatgagcagttgaaatctggaactgcctctgttgtgtgcctgctgaataacttctatcccagagaggccaaagtacagtggaaggtggataacgccctccaatcgggtaactcccaggagagtgtcacagagcaggacagcaaggacagcacctacagcctcagcagcaccctgacgctgagcaaagcagactacgagaaacacaaagtctacgcctgcgaagtcacccatcagggcctgagctcgcccgtcacaaagagcttcaacaggggagagtgttaa

SEQ ID NO: 24 - protein, 215 aa, synthetic construct
  REGION 1..215: note = anti-CD47 Ke8G6 kappa light chain
DIQMTQSPSSLSASVGDRVTITCRASQSIGRYLNWYQQKPGKAPKLLIYAASSLQSGVPSRFSGSGSGTDFTLTISSLQPEDFATYYCQQMHPRAPKTFGQGTKVEIKRTVAAPSVFIFPPSDEQLKSGTASVVCLLNNFYPREAKVQWKVDNALQSGNSQESVTEQDSKDSTYSLSSTLTLSKADYEKHKVYACEVTHQGLSSPVTKSFNRGEC

SEQ ID NO: 25 - DNA, 648 bp, synthetic construct
  misc_feature 1..648: note = anti-CD47 Ke8A3 kappa light chain
  source 1..648: mol_type = other DNA
gacatccagatgacccagtctccatcctccctgtctgcatctgtaggagacagagtcaccatcacttgccgggtaagtcagagcattagtaagtatttaaattggtatcagcagaaaccagggaaagcccctaagctcctgatctatgctgcatccagtttgcaaagtggggtcccatcaaggttcagtggcagtggatctgggacagatttcactctcaccatcagcagtctgcaacctgaagattttgcaacttactactgtcagcagaggcatccccgtgggccgagcaccttcggccaagggaccaaggtggaaatcaaacgtacggtggctgcaccatctgtcttcatcttcccgccatctgatgagcagttgaaatctggaactgcctctgttgtgtgcctgctgaataacttctatcccagagaggccaaagtacagtggaaggtggataacgccctccaatcgggtaactcccaggagagtgtcacagagcaggacagcaaggacagcacctacagcctcagcagcaccctgacgctgagcaaagcagactacgagaaacacaaagtctacgcctgcgaagtcacccatcagggcctgagctcgcccgtcacaaagagcttcaacaggggagagtgttaa

SEQ ID NO: 26 - protein, 215 aa, synthetic construct
  REGION 1..215: note = anti-CD47 Ke8A3 kappa light chain
DIQMTQSPSSLSASVGDRVTITCRVSQSISKYLNWYQQKPGKAPKLLIYAASSLQSGVPSRFSGSGSGTDFTLTISSLQPEDFATYYCQQRHPRGPSTFGQGTKVEIKRTVAAPSVFIFPPSDEQLKSGTASVVCLLNNFYPREAKVQWKVDNALQSGNSQESVTEQDSKDSTYSLSSTLTLSKADYEKHKVYACEVTHQGLSSPVTKSFNRGEC

SEQ ID NO: 27 - DNA, 648 bp, synthetic construct
  misc_feature 1..648: note = anti-CD47 Ke81A3 kappa light chain
  source 1..648: mol_type = other DNA
gacatccagatgacccagtctccatcctccctgtctgcatctgtaggagacagagtcaccatcacttgccaggcgagtcaggacattaataggtatttaaattggtatcagcagaaaccagggaaagcccctaagctcctgatctatgctgcatccagtttgcaaagtggggtcccatcaaggttcagtggcagtggatctgggacagatttcactctcaccatcagcagtctgcaacctgaagattttgcaacttactactgtcagcagaggcatccgcgtgccccgcggaccttcggccaagggaccaaggtggaaatcaaacgtacggtggctgcaccatctgtcttcatcttcccgccatctgatgagcagttgaaatctggaactgcctctgttgtgtgcctgctgaataacttctatcccagagaggccaaagtacagtggaaggtggataacgccctccaatcgggtaactcccaggagagtgtcacagagcaggacagcaaggacagcacctacagcctcagcagcaccctgacgctgagcaaagcagactacgagaaacacaaagtctacgcctgcgaagtcacccatcagggcctgagctcgcccgtcacaaagagcttcaacaggggagagtgttaa

SEQ ID NO: 28 - protein, 215 aa, synthetic construct
  REGION 1..215: note = anti-CD47 Ke81A3 kappa light chain
DIQMTQSPSSLSASVGDRVTITCQASQDINRYLNWYQQKPGKAPKLLIYAASSLQSGVPSRFSGSGSGTDFTLTISSLQPEDFATYYCQQRHPRAPRTFGQGTKVEIKRTVAAPSVFIFPPSDEQLKSGTASVVCLLNNFYPREAKVQWKVDNALQSGNSQESVTEQDSKDSTYSLSSTLTLSKADYEKHKVYACEVTHQGLSSPVTKSFNRGEC

SEQ ID NO: 29 - DNA, 648 bp, synthetic construct
  misc_feature 1..648: note = anti-CD47 Ke8A8 kappa light chain
  source 1..648: mol_type = other DNA
gacatccagatgacccagtctccatcctccctgtctgcatctgtaggagacagagtcaccatcacttgccgggcaagtcagagcattagtaagtatttaaattggtatcagcagaaaccagggaaagcccctaagctcctgatctatgctgcatccactttgcaaagtggggtcccatcaaggttcagtggcagtggatctgggacagatttcactctcaccatcagcagtctgcaacctgaagattttgcaacttactactgtcagcagatgcatccgcgtgcgccgaagaccttcggccaagggaccaaggtggaaatcaaacgtacggtggctgcaccatctgtcttcatcttcccgccatctgatgagcagttgaaatctggaactgcctctgttgtgtgcctgctgaataacttctatcccagagaggccaaagtacagtggaaggtggataacgccctccaatcgggtaactcccaggagagtgtcacagagcaggacagcaaggacagcacctacagcctcagcagcaccctgacgctgagcaaagcagactacgagaaacacaaagtctacgcctgcgaagtcacccatcagggcctgagctcgcccgtcacaaagagcttcaacaggggagagtgttaa

SEQ ID NO: 30 - protein, 215 aa, synthetic construct
  REGION 1..215: note = anti-CD47 Ke8A8 kappa light chain
DIQMTQSPSSLSASVGDRVTITCRASQSISKYLNWYQQKPGKAPKLLIYAASTLQSGVPSRFSGSGSGTDFTLTISSLQPEDFATYYCQQMHPRAPKTFGQGTKVEIKRTVAAPSVFIFPPSDEQLKSGTASVVCLLNNFYPREAKVQWKVDNALQSGNSQESVTEQDSKDSTYSLSSTLTLSKADYEKHKVYACEVTHQGLSSPVTKSFNRGEC

SEQ ID NO: 31 - DNA, 648 bp, synthetic construct
  misc_feature 1..648: note = anti-CD47 Ke8C7 kappa light chain
  source 1..648: mol_type = other DNA
gacatccagatgacccagtctccatcctccctgtctgcatctgtaggagacagagtcaccatcacttgccaggcgagtcaggacattaataggtatttaaattggtatcagcagaaaccagggaaagcccctaagctcctgatctatgctgcatccagtttgcaaagtggggtcccatcaaggttcagtggcagtggatctgggacagatttcactctcaccatcagcagtctgcaacctgaagattttgcaacttactactgtcagcagcgccatccgcgtggcccgaggaccttcggccaagggaccaaggtggaaatcaaacgtacggtggctgcaccatctgtcttcatcttcccgccatctgatgagcagttgaaatctggaactgcctctgttgtgtgcctgctgaataacttctatcccagagaggccaaagtacagtggaaggtggataacgccctccaatcgggtaactcccaggagagtgtcacagagcaggacagcaaggacagcacctacagcctcagcagcaccctgacgctgagcaaagcagactacgagaaacacaaagtctacgcctgcgaagtcacccatcagggcctgagctcgcccgtcacaaagagcttcaacaggggagagtgttaa

SEQ ID NO: 32 - protein, 215 aa, synthetic construct
  REGION 1..215: note = anti-CD47 Ke8C7 kappa light chain
DIQMTQSPSSLSASVGDRVTITCQASQDINRYLNWYQQKPGKAPKLLIYAASSLQSGVPSRFSGSGSGTDFTLTISSLQPEDFATYYCQQRHPRGPRTFGQGTKVEIKRTVAAPSVFIFPPSDEQLKSGTASVVCLLNNFYPREAKVQWKVDNALQSGNSQESVTEQDSKDSTYSLSSTLTLSKADYEKHKVYACEVTHQGLSSPVTKSFNRGEC

SEQ ID NO: 33 - DNA, 648 bp, synthetic construct
  misc_feature 1..648: note = anti-CD47 Ke8G2 kappa light chain
  source 1..648: mol_type = other DNA
gacatccagatgacccagtctccatcctccctgtctgcatctgtaggagacagagtcaccatcacttgccgggcaagtcagagcattggtaggtatttaaattggtatcagcagaaaccagggaaagcccctaagctcctgatctatgcggcatccaggttgcaaagtggggtcccatcaaggttcagtggcagtggatctgggacagatttcactctcaccatcaacagtctgcaacctgaagattttgcaacttactactgtcagcagaagcatccccgtgcgccgaggaccttcggccaagggaccaaggtggaaatcaaacgtacggtggctgcaccatctgtcttcatcttcccgccatctgatgagcagttgaaatctggaactgcctctgttgtgtgcctgctgaataacttctatcccagagaggccaaagtacagtggaaggtggataacgccctccaatcgggtaactcccaggagagtgtcacagagcaggacagcaaggacagcacctacagcctcagcagcaccctgacgctgagcaaagcagactacgagaaacacaaagtctacgcctgcgaagtcacccatcagggcctgagctcgcccgtcacaaagagcttcaacaggggagagtgttaa

SEQ ID NO: 34 - protein, 215 aa, synthetic construct
  REGION 1..215: note = anti-CD47 Ke8G2 kappa light chain
DIQMTQSPSSLSASVGDRVTITCRASQSIGRYLNWYQQKPGKAPKLLIYAASRLQSGVPSRFSGSGSGTDFTLTINSLQPEDFATYYCQQKHPRAPRTFGQGTKVEIKRTVAAPSVFIFPPSDEQLKSGTASVVCLLNNFYPREAKVQWKVDNALQSGNSQESVTEQDSKDSTYSLSSTLTLSKADYEKHKVYACEVTHQGLSSPVTKSFNRGEC

SEQ ID NO: 35 - DNA, 648 bp, synthetic construct
  misc_feature 1..648: note = anti-CD47 Ke81G9 kappa light chain
  source 1..648: mol_type = other DNA
gacatccagatgacccagtctccatcctccctgtctgcatctgtaggagacagagtcaccatcacttgccgggcaagtcagagcattgataagtatttaaattggtatcagcagaaaccagggaaagcccctaagctcctgatctatgcggcatccaggttgcaaagtggggtcccatcaaggttcagtggcagtggatctgggacagatttcactctcaccatcagcagtctgcaacctgaagattttgcaacttactactgtcagcagcggcataagcgttccccgcagaccttcggccaagggaccaaggtggaaatcaaacgtacggtggctgcaccatctgtcttcatcttcccgccatctgatgagcagttgaaatctggaactgcctctgttgtgtgcctgctgaataacttctatcccagagaggccaaagtacagtggaaggtggataacgccctccaatcgggtaactcccaggagagtgtcacagagcaggacagcaaggacagcacctacagcctcagcagcaccctgacgctgagcaaagcagactacgagaaacacaaagtctacgcctgcgaagtcacccatcagggcctgagctcgcccgtcacaaagagcttcaacaggggagagtgttaa

SEQ ID NO: 36 - protein, 215 aa, synthetic construct
  REGION 1..215: note = anti-CD47 Ke81G9 kappa light chain
DIQMTQSPSSLSASVGDRVTITCRASQSIDKYLNWYQQKPGKAPKLLIYAASRLQSGVPSRFSGSGSGTDFTLTISSLQPEDFATYYCQQRHKRSPQTFGQGTKVEIKRTVAAPSVFIFPPSDEQLKSGTASVVCLLNNFYPREAKVQWKVDNALQSGNSQESVTEQDSKDSTYSLSSTLTLSKADYEKHKVYACEVTHQGLSSPVTKSFNRGEC

SEQ ID NO: 37 - DNA, 648 bp, synthetic construct
  misc_feature 1..648: note = anti-CD47 Ke8F2 kappa light chain
  source 1..648: mol_type = other DNA
gacatccagatgacccagtctccatcctccctgtctgcatctgtaggagacagagtcaccatcacttgccgggcaagtcagagcattgataagtatttaaattggtatcagcagaaaccagggaaagcccctaagctcctgatctatgctgcatccagtttgcaaagtggggtcccatcaaggttcagtggcagtggatctgggacagatttcactctcaccatcagcagtctgcaacctgaagattttgcaacttactactgtcagcagaagcatccgcgtgcgccgcggaccttcggccaagggaccaaggtggaaatcaaacgtacggtggctgcaccatctgtcttcatcttcccgccatctgatgagcagttgaaatctggaactgcctctgttgtgtgcctgctgaataacttctatcccagagaggccaaagtacagtggaaggtggataacgccctccaatcgggtaactcccaggagagtgtcacagagcaggacagcaaggacagcacctacagcctcagcagcaccctgacgctgagcaaagcagactacgagaaacacaaagtctacgcctgcgaagtcacccatcagggcctgagctcgcccgtcacaaagagcttcaacaggggagagtgttaa

SEQ ID NO: 38 - protein, 215 aa, synthetic construct
  REGION 1..215: note = anti-CD47 Ke8F2 kappa light chain
DIQMTQSPSSLSASVGDRVTITCRASQSIDKYLNWYQQKPGKAPKLLIYAASSLQSGVPSRFSGSGSGTDFTLTISSLQPEDFATYYCQQKHPRAPRTFGQGTKVEIKRTVAAPSVFIFPPSDEQLKSGTASVVCLLNNFYPREAKVQWKVDNALQSGNSQESVTEQDSKDSTYSLSSTLTLSKADYEKHKVYACEVTHQGLSSPVTKSFNRGEC

SEQ ID NO: 39 - DNA, 648 bp, synthetic construct
  misc_feature 1..648: note = anti-CD47 Ke8B7 kappa light chain
  source 1..648: mol_type = other DNA
gacatccagatgacccagtctccatcctccctgtctgcatctgtaggagacagagtcaccatcacttgccgggcaagtcagagcattgggaagtatttaaattggtatcagcagaaaccagggaaagcccctaagctcctgatctatgctgcatccagtttgcaaagtggggtcccatcaaggttcagtggcagtggatctgggacagatttcactctcaccatcagcagtctgcaacctgaagattttgcaacttactactgtcagcagatgcatccgcgtagcccgaagaccttcggccaagggaccaaggtggaaatcaaacgtacggtggctgcaccatctgtcttcatcttcccgccatctgatgagcagttgaaatctggaactgcctctgttgtgtgcctgctgaataacttctatcccagagaggccaaagtacagtggaaggtggataacgccctccaatcgggtaactcccaggagagtgtcacagagcaggacagcaaggacagcacctacagcctcagcagcaccctgacgctgagcaaagcagactacgagaaacacaaagtctacgcctgcgaagtcacccatcagggcctgagctcgcccgtcacaaagagcttcaacaggggagagtgttaa

SEQ ID NO: 40 - protein, 215 aa, synthetic construct
  REGION 1..215: note = anti-CD47 Ke8B7 kappa light chain
DIQMTQSPSSLSASVGDRVTITCRASQSIGKYLNWYQQKPGKAPKLLIYAASSLQSGVPSRFSGSGSGTDFTLTISSLQPEDFATYYCQQMHPRSPKTFGQGTKVEIKRTVAAPSVFIFPPSDEQLKSGTASVVCLLNNFYPREAKVQWKVDNALQSGNSQESVTEQDSKDSTYSLSSTLTLSKADYEKHKVYACEVTHQGLSSPVTKSFNRGEC

SEQ ID NO: 41 - DNA, 648 bp, synthetic construct
  misc_feature 1..648: note = anti-CD47 Ke8C4 kappa light chain
  source 1..648: mol_type = other DNA
gacatccagatgacccagtctccatcctccctgtctgcatctgtaggagacagagtcaccatcacttgccgggcaagtcagagcattagtaggtatttaaattggtatcagcagaaaccagggaaagcccctaagctcctgatctatgctgcatccaatttgcaaagtggggtcccatcaaggttcagtggcagtggatctgggacagatttcactctcaccatcagcagtctgcaacctgaagattttgcaacttactactgtcagcagatgcatccgcgtgggccgaagaccttcggccaagggaccaaggtggaaatcaaacgtacggtggctgcaccatctgtcttcatcttcccgccatctgatgagcagttgaaatctggaactgcctctgttgtgtgcctgctgaataacttctatcccagagaggccaaagtacagtggaaggtggataacgccctccaatcgggtaactcccaggagagtgtcacagagcaggacagcaaggacagcacctacagcctcagcagcaccctgacgctgagcaaagcagactacgagaaacacaaagtctacgcctgcgaagtcacccatcagggcctgagctcgcccgtcacaaagagcttcaacaggggagagtgttaa

SEQ ID NO: 42 - protein, 215 aa, synthetic construct
  REGION 1..215: note = anti-CD47 Ke8C4 kappa light chain
DIQMTQSPSSLSASVGDRVTITCRASQSISRYLNWYQQKPGKAPKLLIYAASNLQSGVPSRFSGSGSGTDFTLTISSLQPEDFATYYCQQMHPRGPKTFGQGTKVEIKRTVAAPSVFIFPPSDEQLKSGTASVVCLLNNFYPREAKVQWKVDNALQSGNSQESVTEQDSKDSTYSLSSTLTLSKADYEKHKVYACEVTHQGLSSPVTKSFNRGEC

SEQ ID NO: 43 - DNA, 648 bp, synthetic construct
  misc_feature 1..648: note = anti-CD47 Ke8F1 kappa light chain
  source 1..648: mol_type = other DNA
gacatccagatgacccagtctccatcctccctgtctgcatctgtaggagacagagtcaccatcacttgccgggcaagtcagagcattgcttcttatgtaaattggtatcagcagaaaccagggaaagcccctaagctcctgatctatgctgcatccggtttgcaaagtggggtcccatcaaggttcagtggcagtggatctgggacagatttcactctcaccatcagcagtctgcaacctgaagattttgcaacttactactgtcagcagttccataagcgtcggccgcagaccttcggccaagggaccaaggtggaaatcaaacgtacggtggctgcaccatctgtcttcatcttcccgccatctgatgagcagttgaaatctggaactgcctctgttgtgtgcctgctgaataacttctatcccagagaggccaaagtacagtggaaggtggataacgccctccaatcgggtaactcccaggagagtgtcacagagcaggacagcaaggacagcacctacagcctcagcagcaccctgacgctgagcaaagcagactacgagaaacacaaagtctacgcctgcgaagtcacccatcagggcctgagctcgcccgtcacaaagagcttcaacaggggagagtgttaa

SEQ ID NO: 44 - protein, 215 aa, synthetic construct
  REGION 1..215: note = anti-CD47 Ke8F1 kappa light chain
DIQMTQSPSSLSASVGDRVTITCRASQSIASYVNWYQQKPGKAPKLLIYAASGLQSGVPSRFSGSGSGTDFTLTISSLQPEDFATYYCQQFHKRRPQTFGQGTKVEIKRTVAAPSVFIFPPSDEQLKSGTASVVCLLNNFYPREAKVQWKVDNALQSGNSQESVTEQDSKDSTYSLSSTLTLSKADYEKHKVYACEVTHQGLSSPVTKSFNRGEC

SEQ ID NO: 45 - DNA, 648 bp, synthetic construct
  misc_feature 1..648: note = anti-CD47 Ke8G11 kappa light chain
  source 1..648: mol_type = other DNA
gacatccagatgacccagtctccatcctccctgtctgcatctgtaggagacagagtcaccatcacttgccgggcaagtcagagcattgggaggtatttaaattggtatcagcagaaaccagggaaagcccctaagctcctgatctatgctgcatccagtttgcaaagtggggtcccatcaaggttcagtggcagtggatctgggacagatttcactctcaccatcagcagtctgcaacctgaagattttgcaacttactactgtcagcagatgcatccgcgtgggccgaagaccttcggccaagggaccaaggtggaaatcaaacgtacggtggctgcaccatctgtcttcatcttcccgccatctgatgagcagttgaaatctggaactgcctctgttgtgtgcctgctgaataacttctatcccagagaggccaaagtacagtggaaggtggataacgccctccaatcgggtaactcccaggagagtgtcacagagcaggacagcaaggacagcacctacagcctcagcagcaccctgacgctgagcaaagcagactacgagaaacacaaagtctacgcctgcgaagtcacccatcagggcctgagctcgcccgtcacaaagagcttcaacaggggagagtgttaa

SEQ ID NO: 46 - protein, 215 aa, synthetic construct
  REGION 1..215: note = anti-CD47 Ke8G11 kappa light chain
DIQMTQSPSSLSASVGDRVTITCRASQSIGRYLNWYQQKPGKAPKLLIYAASSLQSGVPSRFSGSGSGTDFTLTISSLQPEDFATYYCQQMHPRGPKTFGQGTKVEIKRTVAAPSVFIFPPSDEQLKSGTASVVCLLNNFYPREAKVQWKVDNALQSGNSQESVTEQDSKDSTYSLSSTLTLSKADYEKHKVYACEVTHQGLSSPVTKSFNRGEC

SEQ ID NO: 47 - DNA, 648 bp, synthetic construct
  misc_feature 1..648: note = anti-CD47 Ke8H6 kappa light chain
  source 1..648: mol_type = other DNA
gacatccagatgacccagtctccatcctccctgtctgcatctgtaggagacagagtcaccatcacttgccgggcaagtcagagcattagtaagtatttaaattggtatcagcagaaaccagggaaagcccctaagctcctgatctataatgcatccactttgcaaagtggggtcccatcaaggttcagtggcagtggatctgggacagatttcactctcaccatcagcagtctgcaacctgaagattttgcaacttactactgtcagcagaggcatccgcgtgggccgcgcaccttcggccaagggaccaaggtggaaatcaaacgtacggtggctgcaccatctgtcttcatcttcccgccatctgatgagcagttgaaatctggaactgcctctgttgtgtgcctgctgaataacttctatcccagagaggccaaagtacagtggaaggtggataacgccctccaatcgggtaactcccaggagagtgtcacagagcaggacagcaaggacagcacctacagcctcagcagcaccctgacgctgagcaaagcagactacgagaaacacaaagtctacgcctgcgaagtcacccatcagggcctgagctcgcccgtcacaaagagcttcaacaggggagagtgttaa

SEQ ID NO: 48 - protein, 215 aa, synthetic construct
  REGION 1..215: note = anti-CD47 Ke8H6 kappa light chain
DIQMTQSPSSLSASVGDRVTITCRASQSISKYLNWYQQKPGKAPKLLIYNASTLQSGVPSRFSGSGSGTDFTLTISSLQPEDFATYYCQQRHPRGPRTFGQGTKVEIKRTVAAPSVFIFPPSDEQLKSGTASVVCLLNNFYPREAKVQWKVDNALQSGNSQESVTEQDSKDSTYSLSSTLTLSKADYEKHKVYACEVTHQGLSSPVTKSFNRGEC

SEQ ID NO: 49 - DNA, 648 bp, synthetic construct
  misc_feature 1..648: note = anti-CD47 Ke84G9 kappa light chain
  source 1..648: mol_type = other DNA
gacatccagatgacccagtctccatcctccctgtctgcatctgtaggagacagagtcaccatcacttgccgggcaagtcagagcattagtaagtatttaaattggtatcagcagaaaccagggaaagcccctaagctcctgatctatgctgcatccagtttgcaaagtggggtcccatcaaggttcagtggcagtggatctgggacagatttcactctcaccatcagcagtctgcaacctgaagattttgcaacttactactgtcagcagaagcatccgcgtagcccgcggaccttcggccaagggaccaaggtggaaatcaaacgtacggtggctgcaccatctgtcttcatcttcccgccatctgatgagcagttgaaatctggaactgcctctgttgtgtgcctgctgaataacttctatcccagagaggccaaagtacagtggaaggtggataacgccctccaatcgggtaactcccaggagagtgtcacagagcaggacagcaaggacagcacctacagcctcagcagcaccctgacgctgagcaaagcagactacgagaaacacaaagtctacgcctgcgaagtcacccatcagggcctgagctcgcccgtcacaaagagcttcaacaggggagagtgttaa

SEQ ID NO: 50 - protein, 215 aa, synthetic construct
  REGION 1..215: note = anti-CD47 Ke84G9 kappa light chain
DIQMTQSPSSLSASVGDRVTITCRASQSISKYLNWYQQKPGKAPKLLIYAASSLQSGVPSRFSGSGSGTDFTLTISSLQPEDFATYYCQQKHPRSPRTFGQGTKVEIKRTVAAPSVFIFPPSDEQLKSGTASVVCLLNNFYPREAKVQWKVDNALQSGNSQESVTEQDSKDSTYSLSSTLTLSKADYEKHKVYACEVTHQGLSSPVTKSFNRGEC

SEQ ID NO: 51 - DNA, 648 bp, synthetic construct
  misc_feature 1..648: note = anti-CD47 Ke8A4 kappa light chain
  source 1..648: mol_type = other DNA
gacatccagatgacccagtctccatcctccctgtctgcatctgtaggagacagagtcaccatcacttgccgggcaagtcagagcattgctaagtatttaaattggtatcagcagaaaccagggaaagcccctaagctcctgatctatgctgcatccagtttgcaaagtggggtcccatcaaggttcagtggcagtggatctgggacagatttcactctcaccatcagcagtctgcaacctgaagattttgcaacttactactgtcagcagttccataagcgtagcccgcagaccttcggccaagggaccaaggtggaaatcaaacgtacggtggctgcaccatctgtcttcatcttcccgccatctgatgagcagttgaaatctggaactgcctctgttgtgtgcctgctgaataacttctatcccagagaggccaaagtacagtggaaggtggataacgccctccaatcgggtaactcccaggagagtgtcacagagcaggacagcaaggacagcacctacagcctcagcagcaccctgacgctgagcaaagcagactacgagaaacacaaagtctacgcctgcgaagtcacccatcagggcctgagctcgcccgtcacaaagagcttcaacaggggagagtgttaa

SEQ ID NO: 52 - protein, 215 aa, synthetic construct
  REGION 1..215: note = anti-CD47 Ke8A4 kappa light chain
DIQMTQSPSSLSASVGDRVTITCRASQSIAKYLNWYQQKPGKAPKLLIYAASSLQSGVPSRFSGSGSGTDFTLTISSLQPEDFATYYCQQFHKRSPQTFGQGTKVEIKRTVAAPSVFIFPPSDEQLKSGTASVVCLLNNFYPREAKVQWKVDNALQSGNSQESVTEQDSKDSTYSLSSTLTLSKADYEKHKVYACEVTHQGLSSPVTKSFNRGEC

SEQ ID NO: 53 - DNA, 648 bp, synthetic construct
  misc_feature 1..648: note = anti-CD47 Ke86G9 kappa light chain
  source 1..648: mol_type = other DNA
gacatccagatgacccagtctccatcctccctgtctgcatctgtaggagacagagtcaccatcacttgccgggcaagtcagagcattagtaagtatttaaattggtatcagcagaaaccagggaaagcccctaagctcctgatctataatgcatccaatttgcaaagtggggtcccatcaaggttcagtggcagtggatctgggacagatttcactctcaccatcagcagtctgcaacctgaagattttgcaacttactactgtcagcagaggcatccgcgtgggccgaccaccttcggccaagggaccaaggtggaaatcaaacgtacggtggctgcaccatctgtcttcatcttcccgccatctgatgagcagttgaaatctggaactgcctctgttgtgtgcctgctgaataacttctatcccagagaggccaaagtacagtggaaggtggataacgccctccaatcgggtaactcccaggagagtgtcacagagcaggacagcaaggacagcacctacagcctcagcagcaccctgacgctgagcaaagcagactacgagaaacacaaagtctacgcctgcgaagtcacccatcagggcctgagctcgcccgtcacaaagagcttcaacaggggagagtgttaa

SEQ ID NO: 54 - protein, 215 aa, synthetic construct
  REGION 1..215: note = anti-CD47 Ke86G9 kappa light chain
DIQMTQSPSSLSASVGDRVTITCRASQSISKYLNWYQQKPGKAPKLLIYNASNLQSGVPSRFSGSGSGTDFTLTISSLQPEDFATYYCQQRHPRGPTTFGQGTKVEIKRTVAAPSVFIFPPSDEQLKSGTASVVCLLNNFYPREAKVQWKVDNALQSGNSQESVTEQDSKDSTYSLSSTLTLSKADYEKHKVYACEVTHQGLSSPVTKSFNRGEC

SEQ ID NO: 55 - DNA, 648 bp, synthetic construct
  misc_feature 1..648: note = anti-CD47 Ka3 kappa light chain
  source 1..648: mol_type = other DNA
gacatccagatgacccagtctccatcctccctgtctgcatctgtaggagacagagtcaccatcacttgccgggcaagtcagagcattagcagctatttaaattggtatcagcagaaaccagggaaagcccctaagctcctgatctatgctgcatccagtttgcaaagtggggtcccatcaaggttcagtggcagtggatctgggacagatttcactctcaccatcagcagtctgcaacctgaagattttgcaacttactactgtcagcagatgcacccgcgcgccccgaagaccttcggccaagggaccaaggtggaaatcaaacgtacggtggctgcaccatctgtcttcatcttcccgccatctgatgagcagttgaaatctggaactgcctctgttgtgtgcctgctgaataacttctatcccagagaggccaaagtacagtggaaggtggataacgccctccaatcgggtaactcccaggagagtgtcacagagcaggacagcaaggacagcacctacagcctcagcagcaccctgacgctgagcaaagcagactacgagaaacacaaagtctacgcctgcgaagtcacccatcagggcctgagctcgcccgtcacaaagagcttcaacaggggagagtgttaa

SEQ ID NO: 56 - protein, 215 aa, synthetic construct
  REGION 1..215: note = anti-CD47 Ka3 kappa light chain
DIQMTQSPSSLSASVGDRVTITCRASQSISSYLNWYQQKPGKAPKLLIYAASSLQSGVPSRFSGSGSGTDFTLTISSLQPEDFATYYCQQMHPRAPKTFGQGTKVEIKRTVAAPSVFIFPPSDEQLKSGTASVVCLLNNFYPREAKVQWKVDNALQSGNSQESVTEQDSKDSTYSLSSTLTLSKADYEKHKVYACEVTHQGLSSPVTKSFNRGEC

SEQ ID NO: 57 - DNA, 648 bp, synthetic construct
  misc_feature 1..648: note = anti-CD47 Ka3A2 kappa light chain
  source 1..648: mol_type = other DNA
gacatccagatgacccagtctccatcctccctgtctgcatctgtaggagacagagtcaccatcacttgccgggcaagtcagagcattagtaagtatttaaattggtatcagcagaaaccagggaaagcccctaagctcctgatctatgctgcatccaggttgcaaagtggggtcccatcaaggttcagtggcagtggatctgggacagatttcactctcaccatcagcagtctgcaacctgaagattttgcaacttactactgtcagcagatgcatcctcgctcgccgaaaaccttcggccaagggaccaaggtggaaatcaaacgtacggtggctgcaccatctgtcttcatcttcccgccatctgatgagcagttgaaatctggaactgcctctgttgtgtgcctgctgaataacttctatcccagagaggccaaagtacagtggaaggtggataacgccctccaatcgggtaactcccaggagagtgtcacagagcaggacagcaaggacagcacctacagcctcagcagcaccctgacgctgagcaaagcagactacgagaaacacaaagtctacgcctgcgaagtcacccatcagggcctgagctcgcccgtcacaaagagcttcaacaggggagagtgttaa

SEQ ID NO: 58 - protein, 215 aa, synthetic construct
  REGION 1..215: note = anti-CD47 Ka3A2 kappa light chain
DIQMTQSPSSLSASVGDRVTITCRASQSISKYLNWYQQKPGKAPKLLIYAASRLQSGVPSRFSGSGSGTDFTLTISSLQPEDFATYYCQQMHPRSPKTFGQGTKVEIKRTVAAPSVFIFPPSDEQLKSGTASVVCLLNNFYPREAKVQWKVDNALQSGNSQESVTEQDSKDSTYSLSSTLTLSKADYEKHKVYACEVTHQGLSSPVTKSFNRGEC

SEQ ID NO: 59 - DNA, 648 bp, synthetic construct
  misc_feature 1..648: note = anti-CD47 Ka3H3 kappa light chain
  source 1..648: mol_type = other DNA
gacatccagatgacccagtctccatcctccctgtctgcatctgtaggagacagagtcaccatcacttgccaggcgagtcaggacattgctaagtatttaaattggtatcagcagaaaccagggaaagcccctaagctcctgatctatgctgcatccgctttgcaaagtggggtcccatcaaggttcagtggcagtggatctgggacagatttcactctcaccatcagcagtctgcaacctgaagattttgcaacttactactgtcagcagatgcatcctcgctcgccgaaaaccttcggccaagggaccaaggtggaaatcaaacgtacggtggctgcaccatctgtcttcatcttcccgccatctgatgagcagttgaaatctggaactgcctctgttgtgtgcctgctgaataacttctatcccagagaggccaaagtacagtggaaggtggataacgccctccaatcgggtaactcccaggagagtgtcacagagcaggacagcaaggacagcacctacagcctcagcagcaccctgacgctgagcaaagcagactacgagaaacacaaagtctacgcctgcgaagtcacccatcagggcctgagctcgcccgtcacaaagagcttcaacaggggagagtgttaa

SEQ ID NO: 60 - protein, 215 aa, synthetic construct
  REGION 1..215: note = anti-CD47 Ka3H3 kappa light chain
DIQMTQSPSSLSASVGDRVTITCQASQDIAKYLNWYQQKPGKAPKLLIYAASALQSGVPSRFSGSGSGTDFTLTISSLQPEDFATYYCQQMHPRSPKTFGQGTKVEIKRTVAAPSVFIFPPSDEQLKSGTASVVCLLNNFYPREAKVQWKVDNALQSGNSQESVTEQDSKDSTYSLSSTLTLSKADYEKHKVYACEVTHQGLSSPVTKSFNRGEC

SEQ ID NO: 61 - DNA, 648 bp, synthetic construct
  misc_feature 1..648: note = anti-CD47 Ka3A3 kappa light chain
  source 1..648: mol_type = other DNA
gacatccagatgacccagtctccatcctccctgtctgcatctgtaggagacagagtcaccatcacttgccgggcaagtcagagcattgctagttatttaaattggtatcagcagaaaccagggaaagcccctaagctcctgatctatgcggcatccaggttgcaaagtggggtcccatcaaggttcagtggcagtggatctgggacagatttcactctcaccatcagcagtctgcaacctgaagattttgcaacttactactgtcagcagatgcatcctcgcgcgccgaaaaccttcggccaagggaccaaggtggaaatcaaacgtacggtggctgcaccatctgtcttcatcttcccgccatctgatgagcagttgaaatctggaactgcctctgttgtgtgcctgctgaataacttctatcccagagaggccaaagtacagtggaaggtggataacgccctccaatcgggtaactcccaggagagtgtcacagagcaggacagcaaggacagcacctacagcctcagcagcaccctgacgctgagcaaagcagactacgagaaacacaaagtctacgcctgcgaagtcacccatcagggcctgagctcgcccgtcacaaagagcttcaacaggggagagtgttaa

SEQ ID NO: 62 - protein, 215 aa, synthetic construct
  REGION 1..215: note = anti-CD47 Ka3A3 kappa light chain
DIQMTQSPSSLSASVGDRVTITCRASQSIASYLNWYQQKPGKAPKLLIYAASRLQSGVPSRFSGSGSGTDFTLTISSLQPEDFATYYCQQMHPRAPKTFGQGTKVEIKRTVAAPSVFIFPPSDEQLKSGTASVVCLLNNFYPREAKVQWKVDNALQSGNSQESVTEQDSKDSTYSLSSTLTLSKADYEKHKVYACEVTHQGLSSPVTKSFNRGEC

SEQ ID NO: 63 - DNA, 648 bp, synthetic construct
  misc_feature 1..648: note = anti-CD47 Ka3H8 kappa light chain
  source 1..648: mol_type = other DNA
gacatccagatgacccagtctccatcctccctgtctgcatctgtaggagacagagtcaccatcacttgccgggcaagtcagagcattgcgagttatttaaattggtatcagcagaaaccagggaaagcccctaagctcctgatctatgcggcatccaggttgcaaagtggggtcccatcaaggttcagtggcagtggatctgggacagatttcactctcaccatcagcagtctgcaacctgaagattttgcaacttactactgtcagcagatgcatcctcgctcgccgaaaaccttcggccaagggaccaaggtggaaatcaaacgtacggtggctgcaccatctgtcttcatcttcccgccatctgatgagcagttgaaatctggaactgcctctgttgtgtgcctgctgaataacttctatcccagagaggccaaagtacagtggaaggtggataacgccctccaatcgggtaactcccaggagagtgtcacagagcaggacagcaaggacagcacctacagcctcagcagcaccctgacgctgagcaaagcagactacgagaaacacaaagtctacgcctgcgaagtcacccatcagggcctgagctcgcccgtcacaaagagcttcaacaggggagagtgttaa

SEQ ID NO: 64 - protein, 215 aa, synthetic construct
  REGION 1..215: note = anti-CD47 Ka3H8 kappa light chain
DIQMTQSPSSLSASVGDRVTITCRASQSIASYLNWYQQKPGKAPKLLIYAASRLQSGVPSRFSGSGSGTDFTLTISSLQPEDFATYYCQQMHPRSPKTFGQGTKVEIKRTVAAPSVFIFPPSDEQLKSGTASVVCLLNNFYPREAKVQWKVDNALQSGNSQESVTEQDSKDSTYSLSSTLTLSKADYEKHKVYACEVTHQGLSSPVTKSFNRGEC

SEQ ID NO: 65 - DNA, 648 bp, synthetic construct
  misc_feature 1..648: note = anti-CD47 Ka3B2 kappa light chain
  source 1..648: mol_type = other DNA
gacatccagatgacccagtctccatcctccctgtctgcatctgtaggagacagagtcaccatcacttgccgggcaagtcagaacattggtaagtatttaaattggtatcagcagaaaccagggaaagcccctaagctcctgatctatagtgcatccaggttgcaaagtggggtcccatcaaggttcagtggcagtggatctgggacagatttcactctcaccatcagcagtctgcaacctgaagattttgcaacttactactgtcagcagatgcatcctcgcgcgccgaaaaccttcggccaagggaccaaggtggaaatcaaacgtacggtggctgcaccatctgtcttcatcttcccgccatctgatgagcagttgaaatctggaactgcctctgttgtgtgcctgctgaataacttctatcccagagaggccaaagtacagtggaaggtggataacgccctccaatcgggtaactcccaggagagtgtcacagagcaggacagcaaggacagcacctacagcctcagcagcaccctgacgctgagcaaagcagactacgagaaacacaaagtctacgcctgcgaagtcacccatcagggcctgagctcgcccgtcacaaagagcttcaacaggggagagtgttaa

SEQ ID NO: 66 - protein, 215 aa, synthetic construct
  REGION 1..215: note = anti-CD47 Ka3B2 kappa light chain
DIQMTQSPSSLSASVGDRVTITCRASQNIGKYLNWYQQKPGKAPKLLIYSASRLQSGVPSRFSGSGSGTDFTLTISSLQPEDFATYYCQQMHPRAPKTFGQGTKVEIKRTVAAPSVFIFPPSDEQLKSGTASVVCLLNNFYPREAKVQWKVDNALQSGNSQESVTEQDSKDSTYSLSSTLTLSKADYEKHKVYACEVTHQGLSSPVTKSFNRGEC

SEQ ID NO: 67 - DNA, 648 bp, synthetic construct
  misc_feature 1..648: note = anti-CD47 Ka3C5 kappa light chain
  source 1..648: mol_type = other DNA
gacatccagatgacccagtctccatcctccctgtctgcatctgtaggagacagagtcaccatcacttgccgggcaagtcagagcattagtaggtatttaaattggtatcagcagaaaccagggaaagcccctaagctcctgatctattctgcatcctctttgcaaagtggggtcccatcaaggttcagtggcagtggatctgggacagatttcactctcaccatcagcagtctgcaacctgaagattttgcaacttactactgtcagcagatgcatcctcgcgccccgaaaaccttcggccaagggaccaaggtggaaatcaaacgtacggtggctgcaccatctgtcttcatcttcccgccatctgatgagcagttgaaatctggaactgcctctgttgtgtgcctgctgaataacttctatcccagagaggccaaagtacagtggaaggtggataacgccctccaatcgggtaactcccaggagagtgtcacagagcaggacagcaaggacagcacctacagcctcagcagcaccctgacgctgagcaaagcagactacgagaaacacaaagtctacgcctgcgaagtcacccatcagggcctgagctcgcccgtcacaaagagcttcaacaggggagagtgttaa

SEQ ID NO: 68 - protein, 215 aa, synthetic construct
  REGION 1..215: note = anti-CD47 Ka3C5 kappa light chain
DIQMTQSPSSLSASVGDRVTITCRASQSISRYLNWYQQKPGKAPKLLIYSASSLQSGVPSRFSGSGSGTDFTLTISSLQPEDFATYYCQQMHPRAPKTFGQGTKVEIKRTVAAPSVFIFPPSDEQLKSGTASVVCLLNNFYPREAKVQWKVDNALQSGNSQESVTEQDSKDSTYSLSSTLTLSKADYEKHKVYACEVTHQGLSSPVTKSFNRGEC

SEQ ID NO: 69 - DNA, 648 bp, synthetic construct
  misc_feature 1..648: note = anti-CD47 Ka3G2 kappa light chain
  source 1..648: mol_type = other DNA
gacatccagatgacccagtctccatcctccctgtctgcatctgtaggagacagagtcaccatcacttgccgggcaagtcagagcattgataagtatttaaattggtatcagcagaaaccagggaaagcccctaagctcctgatctatgctgcatccaggttgcaaagtggggtcccatcaaggttcagtggcagtggatctgggacagatttcactctcaccatcagcagtctgcaacctgaagattttgcaacttactactgtcagcagatgcatcctcgcgggccgaaaaccttcggccaagggaccaaggtggaaatcaaacgtacggtggctgcaccatctgtcttcatcttcccgccatctgatgagcagttgaaatctggaactgcctctgttgtgtgcctgctgaataacttctatcccagagaggccaaagtacagtggaaggtggataacgccctccaatcgggtaactcccaggagagtgtcacagagcaggacagcaaggacagcacctacagcctcagcagcaccctgacgctgagcaaagcagactacgagaaacacaaagtctacgcctgcgaagtcacccatcagggcctgagctcgcccgtcacaaagagcttcaacaggggagagtgttaa

SEQ ID NO: 70 - protein, 215 aa, synthetic construct
  REGION 1..215: note = anti-CD47 Ka3G2 kappa light chain
DIQMTQSPSSLSASVGDRVTITCRASQSIDKYLNWYQQKPGKAPKLLIYAASRLQSGVPSRFSGSGSGTDFTLTISSLQPEDFATYYCQQMHPRGPKTFGQGTKVEIKRTVAAPSVFIFPPSDEQLKSGTASVVCLLNNFYPREAKVQWKVDNALQSGNSQESVTEQDSKDSTYSLSSTLTLSKADYEKHKVYACEVTHQGLSSPVTKSFNRGEC

SEQ ID NO: 71 - DNA, 648 bp, synthetic construct
  misc_feature 1..648: note = anti-CD47 Ka3D3 kappa light chain
  source 1..648: mol_type = other DNA
gacatccagatgacccagtctccatcctccctgtctgcatctgtaggagacagagtcaccatcacttgccgggcaagtcagagcattggtaagtatttaaattggtatcagcagaaaccagggaaagcccctaagctcctgatctatgctgcatccaggttgcaaagtggggtcccatcaaggttcagtggcagtggatctgggacagatttcactctcaccatcagcagtctgcaacctgaagattttgcaacttactactgtcagcagatgcatcctcgcgcgccgaaaaccttcggccaagggaccaaggtggaaatcaaacgtacggtggctgcaccatctgtcttcatcttcccgccatctgatgagcagttgaaatctggaactgcctctgttgtgtgcctgctgaataacttctatcccagagaggccaaagtacagtggaaggtggataacgccctccaatcgggtaactcccaggagagtgtcacagagcaggacagcaaggacagcacctacagcctcagcagcaccctgacgctgagcaaagcagactacgagaaacacaaagtctacgcctgcgaagtcacccatcagggcctgagctcgcccgtcacaaagagcttcaacaggggagagtgttaa

SEQ ID NO: 72 - protein, 215 aa, synthetic construct
  REGION 1..215: note = anti-CD47 Ka3D3 kappa light chain
DIQMTQSPSSLSASVGDRVTITCRASQSIGKYLNWYQQKPGKAPKLLIYAASRLQSGVPSRFSGSGSGTDFTLTISSLQPEDFATYYCQQMHPRAPKTFGQGTKVEIKRTVAAPSVFIFPPSDEQLKSGTASVVCLLNNFYPREAKVQWKVDNALQSGNSQESVTEQDSKDSTYSLSSTLTLSKADYEKHKVYACEVTHQGLSSPVTKSFNRGEC

SEQ ID NO: 73 - DNA, 654 bp, synthetic construct
  misc_feature 1..654: note = anti-CD47 Kc4 kappa light chain
  source 1..654: mol_type = other DNA
cagtctgccctgactcagcctgcctccgtgtctgggtctcctggacagtcgatcaccatctcctgcactggaaccagcagtgacgttggtggttataactatgtctcctggtaccaacagcacccaggcaaagcccccaaactcatgatttatgaggtcagtaatcggccctcaggggtttctaatcgcttctctggctccaagtctggcaacacggcctccctgaccatctctgggctccaggctgaggacgaggctgattattactgcagctcatatgattggtggttccgccccaaggtgttcggcggagggaccaagctgaccgtcctaggtcagcccaaggctgccccctcggtcactctgttcccgccctcctctgaggagcttcaagccaacaaggccacactggtgtgtctcataagtgacttctacccgggagccgtgacagtggcttggaaagcagatagcagccccgtcaaggcgggagtggagaccaccacaccctccaaacaaagcaacaacaagtacgcggccagcagctatctgagcctgacgcctgagcagtggaagtcccacagaagctacagctgccaggtcacgcatgaagggagcaccgtggagaagacagtggcccctacagaatgttcataa

SEQ ID NO: 74 - protein, 217 aa, synthetic construct
  REGION 1..217: note = anti-CD47 Kc4 kappa light chain
QSALTQPASVSGSPGQSITISCTGTSSDVGGYNYVSWYQQHPGKAPKLMIYEVSNRPSGVSNRFSGSKSGNTASLTISGLQAEDEADYYCSSYDWWFRPKVFGGGTKLTVLGQPKAAPSVTLFPPSSEELQANKATLVCLISDFYPGAVTVAWKADSSPVKAGVETTTPSKQSNNKYAASSYLSLTPEQWKSHRSYSCQVTHEGSTVEKTVAPTECS

SEQ ID NO: 75 - DNA, 654 bp, synthetic construct
  misc_feature 1..654: note = anti-CD47 Kc4G11 kappa light chain
  source 1..654: mol_type = other DNA
cagtctgccctgactcagcctgcctccgtgtctgggtctcctggacagtcgatcaccatctcctgcactggaaccagcagtgacgttgggaaggcgaactatgtctcctggtaccaacagcacccaggcaaagcccccaaactcatgatttataaggatagtgatcggccctcaggggtttctaatcgcttctctggctccaagtctggcaacacggcctccctgaccatctctgggctccaggctgaggacgaggctgattattactgcagctcatatgattggtggttccgccccaaggtgttcggcggagggaccaagctgaccgtcctaggtcagcccaaggctgccccctcggtcactctgttcccgccctcctctgaggagcttcaagccaacaaggccacactggtgtgtctcataagtgacttctacccgggagccgtgacagtggcttggaaagcagatagcagccccgtcaaggcgggagtggagaccaccacaccctccaaacaaagcaacaacaagtacgcggccagcagctatctgagcctgacgcctgagcagtggaagtcccacagaagctacagctgccaggtcacgcatgaagggagcaccgtggagaagacagtggcccctacagaatgttcataa

SEQ ID NO: 76 - protein, 217 aa, synthetic construct
  REGION 1..217: note = anti-CD47 Kc4G11 kappa light chain
QSALTQPASVSGSPGQSITISCTGTSSDVGKANYVSWYQQHPGKAPKLMIYKDSDRPSGVSNRFSGSKSGNTASLTISGLQAEDEADYYCSSYDWWFRPKVFGGGTKLTVLGQPKAAPSVTLFPPSSEELQANKATLVCLISDFYPGAVTVAWKADSSPVKAGVETTTPSKQSNNKYAASSYLSLTPEQWKSHRSYSCQVTHEGSTVEKTVAPTECS

SEQ ID NO: 77 - DNA, 654 bp, synthetic construct
  misc_feature 1..654: note = anti-CD47 Kc4C11 kappa light chain
  source 1..654: mol_type = other DNA
cagtctgccctgactcagcctgcctccgtgtctgggtctcctggacagtcgatcaccatctcctgcactggaaccagcagtgacgttagggggaataactatgtctcctggtaccaacagcacccaggcaaagcccccaaactcatgatttatgagaatagtaagcggccctcaggggtttctaatcgcttctctggctccaagtctggcaacacggcctccctgaccatctctgggctccaggctgaggacgaggctgattattactgcagctcatatgattggtggttccgccccaaggtgttcggcggagggaccaagctgaccgtcctaggtcagcccaaggctgccccctcggtcactctgttcccgccctcctctgaggagcttcaagccaacaaggccacactggtgtgtctcataagtgacttctacccgggagccgtgacagtggcttggaaagcagatagcagccccgtcaaggcgggagtggagaccaccacaccctccaaacaaagcaacaacaagtacgcggccagcagctatctgagcctgacgcctgagcagtggaagtcccacagaagctacagctgccaggtcacgcatgaagggagcaccgtggagaagacagtggcccctacagaatgttcataa

SEQ ID NO: 78 - protein, 217 aa, synthetic construct
  REGION 1..217: note = anti-CD47 Kc4C11 kappa light chain
QSALTQPASVSGSPGQSITISCTGTSSDVRGNNYVSWYQQHPGKAPKLMIYENSKRPSGVSNRFSGSKSGNTASLTISGLQAEDEADYYCSSYDWWFRPKVFGGGTKLTVLGQPKAAPSVTLFPPSSEELQANKATLVCLISDFYPGAVTVAWKADSSPVKAGVETTTPSKQSNNKYAASSYLSLTPEQWKSHRSYSCQVTHEGSTVEKTVAPTECS

SEQ ID NO: 79 - DNA, 654 bp, synthetic construct
  misc_feature 1..654: note = anti-CD47 Kc4A1 kappa light chain
  source 1..654: mol_type = other DNA
cagtctgccctgactcagcctgcctccgtgtctgggtctcctggacagtcgatcaccatctcctgcactggaaccagcagtgacgttagtgcgaggaactatgtctcctggtaccaacagcacccaggcaaagcccccaaactcatgatttatgagagtagtaagcggccctcaggggtttctaatcgcttctctggctccaagtctggcaacacggcctccctgaccatctctgggctccaggctgaggacgaggctgattattactgcagctcatatgattggtggttccgccccaaggtgttcggcggagggaccaagctgaccgtcctaggtcagcccaaggctgccccctcggtcactctgttcccgccctcctctgaggagcttcaagccaacaaggccacactggtgtgtctcataagtgacttctacccgggagccgtgacagtggcttggaaagcagatagcagccccgtcaaggcgggagtggagaccaccacaccctccaaacaaagcaacaacaagtacgcggccagcagctatctgagcctgacgcctgagcagtggaagtcccacagaagctacagctgccaggtcacgcatgaagggagcaccgtggagaagacagtggcccctacagaatgttcataa

SEQ ID NO: 80 - protein, 217 aa, synthetic construct
  REGION 1..217: note = anti-CD47 Kc4A1 kappa light chain
QSALTQPASVSGSPGQSITISCTGTSSDVSARNYVSWYQQHPGKAPKLMIYESSKRPSGVSNRFSGSKSGNTASLTISGLQAEDEADYYCSSYDWWFRPKVFGGGTKLTVLGQPKAAPSVTLFPPSSEELQANKATLVCLISDFYPGAVTVAWKADSSPVKAGVETTTPSKQSNNKYAASSYLSLTPEQWKSHRSYSCQVTHEGSTVEKTVAPTECS

SEQ ID NO: 81 - DNA, 654 bp, synthetic construct
  misc_feature 1..654: note = anti-CD47 Kc4A4 kappa light chain
  source 1..654: mol_type = other DNA
cagtctgccctgactcagcctgcctccgtgtctgggtctcctggacagtcgatcaccatctcctgcactagaaccagcagtgacgttaataatactaactatgtctcctggtaccaacagcacccaggcaaagcccccaaactcatgatttataagactagtggtcggccctcaggggtttctaatcgcttctctggctccaagtctggcaacacggcctccctgaccatctctgggctccaggctgaggacgaggctgattattactgcagctcatatgattggtggttccgccccaaggtgttcggcggagggaccaagctgaccgtcctaggtcagcccaaggctgccccctcggtcactctgttcccgccctcctctgaggagcttcaagccaacaaggccacactggtgtgtctcataagtgacttctacccgggagccgtgacagtggcttggaaagcagatagcagccccgtcaaggcgggagtggagaccaccacaccctccaaacaaagcaacaacaagtacgcggccagcagctatctgagcctgacgcctgagcagtggaagtcccacagaagctacagctgccaggtcacgcatgaagggagcaccgtggagaagacagtggcccctacagaatgttcataa

SEQ ID NO: 82 - protein, 217 aa, synthetic construct
  REGION 1..217: note = anti-CD47 Kc4A4 kappa light chain
QSALTQPASVSGSPGQSITISCTRTSSDVNNTNYVSWYQQHPGKAPKLMIYKTSGRPSGVSNRFSGSKSGNTASLTISGLQAEDEADYYCSSYDWWFRPKVFGGGTKLTVLGQPKAAPSVTLFPPSSEELQANKATLVCLISDFYPGAVTVAWKADSSPVKAGVETTTPSKQSNNKYAASSYLSLTPEQWKSHRSYSCQVTHEGSTVEKTVAPTECS

SEQ ID NO: 83 - DNA, 654 bp, synthetic construct
  misc_feature 1..654: note = anti-CD47 Kc4E10 kappa light chain
  source 1..654: mol_type = other DNA
cagtctgccctgactcagcctgcctccgtgtctgggtctcctggacagtcgatcaccatctcctgcactggaaccagcagtgacgttaattctgctaactatgtctcctggtaccaacagcacccaggcaaagcccccaaactcatgatttataagagtagtagtcggccctcaggggtttctaatcgcttctctggctccaagtctggcaacacggcctccctgaccatctctgggctccaggctgaggacgaggctgattattactgcagctcatatgattggtggttccgccccaaggtgttcggcggagggaccaagctgaccgtcctaggtcagcccaaggctgccccctcggtcactctgttcccgccctcctctgaggagcttcaagccaacaaggccacactggtgtgtctcataagtgacttctacccgggagccgtgacagtggcttggaaagcagatagcagccccgtcaaggcgggagtggagaccaccacaccctccaaacaaagcaacaacaagtacgcggccagcagctatctgagcctgacgcctgagcagtggaagtcccacagaagctacagctgccaggtcacgcatgaagggagcaccgtggagaagacagtggcccctacagaatgttcataa

SEQ ID NO: 84 - protein, 217 aa, synthetic construct
  REGION 1..217: note = anti-CD47 Kc4E10 kappa light chain
QSALTQPASVSGSPGQSITISCTGTSSDVNSANYVSWYQQHPGKAPKLMIYKSSSRPSGVSNRFSGSKSGNTASLTISGLQAEDEADYYCSSYDWWFRPKVFGGGTKLTVLGQPKAAPSVTLFPPSSEELQANKATLVCLISDFYPGAVTVAWKADSSPVKAGVETTTPSKQSNNKYAASSYLSLTPEQWKSHRSYSCQVTHEGSTVEKTVAPTECS

SEQ ID NO: 85 - DNA, 654 bp, synthetic construct
  misc_feature 1..654: note = anti-CD47 Kc4G9 kappa light chain
  source 1..654: mol_type = other DNA
cagtctgccctgactcagcctgcctccgtgtccgggtctcctggacagtcgatcaccatctcctgcactggaaccagcagtgacgttgagaggaagaactatgtctcctggtaccaacagcacccaggcaaagcccccaaactcatgatttataagaatagtactcggccctcaggggtttctaatcgcttctctggctccaagtctggcaacacggcctccctgaccatctctgggctccaggctgaggacgaggctgattattactgcagctcatatgattggtggttccgccccaaggtgttcggcggagggaccaagctgaccgtcctaggtcagcccaaggctgccccctcggtcactctgttcccgccctcctctgaggagcttcaagccaacaaggccacactggtgtgtctcataagtgacttctacccgggagccgtgacagtggcttggaaagcagatagcagccccgtcaaggcgggagtggagaccaccacaccctccaaacaaagcaacaacaagtacgcggccagcagctatctgagcctgacgcctgagcagtggaagtcccacagaagctacagctgccaggtcacgcatgaagggagcaccgtggagaagacagtggcccctacagaatgttcataa

SEQ ID NO: 86 - protein, 217 aa, synthetic construct
  REGION 1..217: note = anti-CD47 Kc4G9 kappa light chain
QSALTQPASVSGSPGQSITISCTGTSSDVERKNYVSWYQQHPGKAPKLMIYKNSTRPSGVSNRFSGSKSGNTASLTISGLQAEDEADYYCSSYDWWFRPKVFGGGTKLTVLGQPKAAPSVTLFPPSSEELQANKATLVCLISDFYPGAVTVAWKADSSPVKAGVETTTPSKQSNNKYAASSYLSLTPEQWKSHRSYSCQVTHEGSTVEKTVAPTECS

SEQ ID NO: 87 - DNA, 654 bp, synthetic construct
  misc_feature 1..654: note = anti-CD47 Kc4C3 kappa light chain
  source 1..654: mol_type = other DNA
cagtctgccctgactcagcctgcctccgtgtctgggtctcctggacagtcgatcaccatctcctgcactggaaccagcagtgacgttagggcggctaactatgtctcctggtaccaacagcacccaggcaaagcccccaaactcatgatttataagaatagtactcggccctcaggggtttctaatcgcttctctggctccaagtctggcaacacggcctccctgaccatctctgggctccaggctgaggacgaggctgattattactgcagctcatatgattggtggttccgccccaaggtgttcggcggagggaccaagctgaccgtcctaggtcagcccaaggctgccccctcggtcactctgttcccgccctcctctgaggagcttcaagccaacaaggccacactggtgtgtctcataagtgacttctacccgggagccgtgacagtggcttggaaagcagatagcagccccgtcaaggcgggagtggagaccaccacaccctccaaacaaagcaacaacaagtacgcggccagcagctatctgagcctgacgcctgagcagtggaagtcccacagaagctacagctgccaggtcacgcatgaagggagcaccgtggagaagacagtggcccctacagaatgttcataa

SEQ ID NO: 88 - protein, 217 aa, synthetic construct
  REGION 1..217: note = anti-CD47 Kc4C3 kappa light chain
QSALTQPASVSGSPGQSITISCTGTSSDVRAANYVSWYQQHPGKAPKLMIYKNSTRPSGVSNRFSGSKSGNTASLTISGLQAEDEADYYCSSYDWWFRPKVFGGGTKLTVLGQPKAAPSVTLFPPSSEELQANKATLVCLISDFYPGAVTVAWKADSSPVKAGVETTTPSKQSNNKYAASSYLSLTPEQWKSHRSYSCQVTHEGSTVEKTVAPTECS

SEQ ID NO: 89 - DNA, 654 bp, synthetic construct
  misc_feature 1..654: note = anti-CD47 Kc4F4 kappa light chain
  source 1..654: mol_type = other DNA
cagtctgccctgactcagcctgcctccgtgtctgggtctcctggacagtcgatcaccatctcctgcactggaaccagcagtgacgttaggagggctaactatgtctcctggtaccaacagcacccaggcaaagcccccaaactcatgatttatcaggatagtagtcggccctcaggggtttctaatcgcttctctggctccaagtctggcaacacggcctccctgaccatctctgggctccaggctgaggacgaggctgattattactgcagctcatatgattggtggttccgccccaaggtgttcggcggagggaccaagctgaccgtcctaggtcagcccaaggctgccccctcggtcactctgttcccgccctcctctgaggagcttcaagccaacaaggccacactggtgtgtctcataagtgacttctacccgggagccgtgacagtggcttggaaagcagatagcagccccgtcaaggcgggagtggagaccaccacaccctccaaacaaagcaacaacaagtacgcggccagcagctatctgagcctgacgcctgagcagtggaagtcccacagaagctacagctgccaggtcacgcatgaagggagcaccgtggagaagacagtggcccctacagaatgttcataa

SEQ ID NO: 90 - protein, 217 aa, synthetic construct
  REGION 1..217: note = anti-CD47 Kc4F4 kappa light chain
QSALTQPASVSGSPGQSITISCTGTSSDVRRANYVSWYQQHPGKAPKLMIYQDSSRPSGVSNRFSGSKSGNTASLTISGLQAEDEADYYCSSYDWWFRPKVFGGGTKLTVLGQPKAAPSVTLFPPSSEELQANKATLVCLISDFYPGAVTVAWKADSSPVKAGVETTTPSKQSNNKYAASSYLSLTPEQWKSHRSYSCQVTHEGSTVEKTVAPTECS

SEQ ID NO: 91 - DNA, 654 bp, synthetic construct
  misc_feature 1..654: note = anti-CD47 Kc4B1 kappa light chain
  source 1..654: mol_type = other DNA
cagtctgccctgactcagcctgcctccgtgtctgggtctcctggacagtcgatcaccatctcctgcactggaaccagcagtgacgttagggctaataactatgtctcctggtaccaacagcacccaggcaaagcccccaaactcatgatttatgagagtagtgcgcggccctcaggggtttctaatcgcttctctggctccaagtctggcaacacggcctccctgaccatctctgggctccaggctgaggacgaggctgattattactgcagctcatatgattggtggttccgccccaaggtgttcggcggagggaccaagctgaccgtcctaggtcagcccaaggctgccccctcggtcactctgttcccgccctcctctgaggagcttcaagccaacaaggccacactggtgtgtctcataagtgacttctacccgggagccgtgacagtggcttggaaagcagatagcagccccgtcaaggcgggagtggagaccaccacaccctccaaacaaagcaacaacaagtacgcggccagcagctatctgagcctgacgcctgagcagtggaagtcccacagaagctacagctgccaggtcacgcatgaagggagcaccgtggagaagacagtggcccctacagaatgttcataa

SEQ ID NO: 92 - protein, 217 aa, synthetic construct
  REGION 1..217: note = anti-CD47 Kc4B1 kappa light chain
QSALTQPASVSGSPGQSITISCTGTSSDVRANNYVSWYQQHPGKAPKLMIYESSARPSGVSNRFSGSKSGNTASLTISGLQAEDEADYYCSSYDWWFRPKVFGGGTKLTVLGQPKAAPSVTLFPPSSEELQANKATLVCLISDFYPGAVTVAWKADSSPVKAGVETTTPSKQSNNKYAASSYLSLTPEQWKSHRSYSCQVTHEGSTVEKTVAPTECS

SEQ ID NO: 93 - DNA, 654 bp, synthetic construct
  misc_feature 1..654: note = anti-CD47 Kc4E2 kappa light chain
  source 1..654: mol_type = other DNA
cagtctgccctgactcagcctgcctccgtgtctgggtctcctggacagtcgatcaccatctcctgcactggaaccagcagtgacgtttattataataagtatgtctcctggtaccaacagcacccaggcaaagcccccaaactcatgatttatgagagtagtaagcggccctcaggggtttctaatcgcttctctggctccaagtctggcaacacggcctccctgaccatctctgggctccaggctgaggacgaggctgattattactgcagctcatatgattggtggttccgccccaaggtgttcggcggagggaccaagctgaccgtcctaggtcagcccaaggctgccccctcggtcactctgttcccgccctcctctgaggagcttcaagccaacaaggccacactggtgtgtctcataagtgacttctacccgggagccgtgacagtggcttggaaagcagatagcagccccgtcaaggcgggagtggagaccaccacaccctccaaacaaagcaacaacaagtacgcggccagcagctatctgagcctgacgcctgagcagtggaagtcccacagaagctacagctgccaggtcacgcatgaagggagcaccgtggagaagacagtggcccctacagaatgttcataa

SEQ ID NO: 94 - protein, 217 aa, synthetic construct
  REGION 1..217: note = anti-CD47 Kc4E2 kappa light chain
QSALTQPASVSGSPGQSITISCTGTSSDVYYNKYVSWYQQHPGKAPKLMIYESSKRPSGVSNRFSGSKSGNTASLTISGLQAEDEADYYCSSYDWWFRPKVFGGGTKLTVLGQPKAAPSVTLFPPSSEELQANKATLVCLISDFYPGAVTVAWKADSSPVKAGVETTTPSKQSNNKYAASSYLSLTPEQWKSHRSYSCQVTHEGSTVEKTVAPTECS

SEQ ID NO: 95 - DNA, 657 bp, synthetic construct
  misc_feature 1..657: note = anti-CD19 C2 lambda light chain
  source 1..657: mol_type = other DNA
aattttatgctgactcagccccactctgtgtcggagtctccggggaagacggtaaccatctcctgcacccgcagcagtggctctatcgaagataagtatgtgcagtggtaccagcagcgcccgggcagttcccccaccattgtgatctattatgataacgaaagaccctctggggtccctgatcggttctctggctccatcgacagctcctccaactctgcctccctcaccatctctggactgaagactgaggacgaggctgactactactgtcagacctacgaccagagcctgtatggttgggtgttcggcggagggaccaagctgaccgtcctaggtcagcccaaggctgccccctcggtcactctgttcccgccctcctctgaggagcttcaagccaacaaggccacactggtgtgtctcataagtgacttctacccgggagccgtgacagtggcttggaaagcagatagcagccccgtcaaggcgggagtggagaccaccacaccctccaaacaaagcaacaacaagtacgcggccagcagctatctgagcctgacgcctgagcagtggaagtcccacagaagctacagctgccaggtcacgcatgaagggagcaccgtggagaagacagtggcccctacagaatgttcataa

SEQ ID NO: 96 - protein, 218 aa, synthetic construct
  REGION 1..218: note = anti-CD19 C2 lambda light chain
NFMLTQPHSVSESPGKTVTISCTRSSGSIEDKYVQWYQQRPGSSPTIVIYYDNERPSGVPDRFSGSIDSSSNSASLTISGLKTEDEADYYCQTYDQSLYGWVFGGGTKLTVLGQPKAAPSVTLFPPSSEELQANKATLVCLISDFYPGAVTVAWKADSSPVKAGVETTTPSKQSNNKYAASSYLSLTPEQWKSHRSYSCQVTHEGSTVEKTVAPTECS

SEQ ID NO: 97 - DNA, 657 bp, synthetic construct
  misc_feature 1..657: note = anti-CD19 A6 lambda light chain
  source 1..657: mol_type = other DNA
aattttatgctgactcagccccactctgtgtcggagtctccggggaagacggtaaccatctcctgcacccgcagcagtggctctatcggtgataagtatgtgcagtggtaccagcagcgcccgggcagttcccccaccattgtgatctattatgataacgaaagaccctctggggtccctgatcggttctctggctccatcgacagctcctccaactctgcctccctcaccatctctggactgaagactgaggacgaggctgactactactgtcagacgtacgacgagagcctgtatggttgggtgttcggcggagggaccaagctgaccgtcctaggtcagcccaaggctgccccctcggtcactctgttcccgccctcctctgaggagcttcaagccaacaaggccacactggtgtgtctcataagtgacttctacccgggagccgtgacagtggcttggaaagcagatagcagccccgtcaaggcgggagtggagaccaccacaccctccaaacaaagcaacaacaagtacgcggccagcagctatctgagcctgacgcctgagcagtggaagtcccacagaagctacagctgccaggtcacgcatgaagggagcaccgtggagaagacagtggcccctacagaatgttcataa

SEQ ID NO: 98 - protein, 218 aa, synthetic construct
  REGION 1..218: note = anti-CD19 A6 lambda light chain
NFMLTQPHSVSESPGKTVTISCTRSSGSIGDKYVQWYQQRPGSSPTIVIYYDNERPSGVPDRFSGSIDSSSNSASLTISGLKTEDEADYYCQTYDESLYGWVFGGGTKLTVLGQPKAAPSVTLFPPSSEELQANKATLVCLISDFYPGAVTVAWKADSSPVKAGVETTTPSKQSNNKYAASSYLSLTPEQWKSHRSYSCQVTHEGSTVEKTVAPTECS

SEQ ID NO: 99 - DNA, 657 bp, synthetic construct
  misc_feature 1..657: note = anti-CD19 C6 lambda light chain
  source 1..657: mol_type = other DNA
aattttatgctgactcagccccactctgtgtcggagtctccggggaagacggtaaccatctcctgcacccgcagcagtggctctatcaatgataagtatgtgcagtggtaccagcagcgcccgggcagttcccccaccattgtgatctattttgataacgaaagaccctctggggtccctgatcggttctctggctccatcgacagctcctccaactctgcctccctcaccatctctggactgaagactgaggacgaggctgactactactgtcagacctacgacaccagcctgtatggttgggtgttcggcggagggaccaagctgaccgtcctaggtcagcccaaggctgccccctcggtcactctgttcccgccctcctctgaggagcttcaagccaacaaggccacactggtgtgtctcataagtgacttctacccgggagccgtgacagtggcttggaaagcagatagcagccccgtcaaggcgggagtggagaccaccacaccctccaaacaaagcaacaacaagtacgcggccagcagctatctgagcctgacgcctgagcagtggaagtcccacagaagctacagctgccaggtcacgcatgaagggagcaccgtggagaagacagtggcccctacagaatgttcataa

SEQ ID NO: 100 - protein, 218 aa, synthetic construct
  REGION 1..218: note = anti-CD19 C6 lambda light chain
NFMLTQPHSVSESPGKTVTISCTRSSGSINDKYVQWYQQRPGSSPTIVIYFDNERPSGVPDRFSGSIDSSSNSASLTISGLKTEDEADYYCQTYDTSLYGWVFGGGTKLTVLGQPKAAPSVTLFPPSSEELQANKATLVCLISDFYPGAVTVAWKADSSPVKAGVETTTPSKQSNNKYAASSYLSLTPEQWKSHRSYSCQVTHEGSTVEKTVAPTECS

SEQ ID NO: 101 - DNA, 657 bp, synthetic construct
  misc_feature 1..657: note = anti-CD19 C9 lambda light chain
  source 1..657: mol_type = other DNA
aattttatgctgactcagccccactctgtgtcggagtctccggggaagacggtaaccatctcctgcacccgcagcagtggctctatcgctgataagtatgtgcagtggtaccagcagcgcccgggcagttcccccaccattgtgatctattatgataacgaaagaccctctggggtccctgatcggttctctggctccatcgacagctcctccaactctgcctccctcaccatctctggactgaagactgaggacgaggctgactactactgtcagacctacgacgagagcctgtatggttgggtgttcggcggagggaccaagctgaccgtcctaggtcagcccaaggctgccccctcggtcactctgttcccgccctcctctgaggagcttcaagccaacaaggccacactggtgtgtctcataagtgacttctacccgggagccgtgacagtggcttggaaagcagatagcagccccgtcaaggcgggagtggagaccaccacaccctccaaacaaagcaacaacaagtacgcggccagcagctatctgagcctgacgcctgagcagtggaagtcccacagaagctacagctgccaggtcacgcatgaagggagcaccgtggagaagacagtggcccctacagaatgttcataa

SEQ ID NO: 102 - protein, 218 aa, synthetic construct
  REGION 1..218: note = anti-CD19 C9 lambda light chain
NFMLTQPHSVSESPGKTVTISCTRSSGSIADKYVQWYQQRPGSSPTIVIYYDNERPSGVPDRFSGSIDSSSNSASLTISGLKTEDEADYYCQTYDESLYGWVFGGGTKLTVLGQPKAAPSVTLFPPSSEELQANKATLVCLISDFYPGAVTVAWKADSSPVKAGVETTTPSKQSNNKYAASSYLSLTPEQWKSHRSYSCQVTHEGSTVEKTVAPTECS

SEQ ID NO: 103 - DNA, 657 bp, synthetic construct
  misc_feature 1..657: note = anti-CD19 B11 lambda light chain
  source 1..657: mol_type = other DNA
aattttatgctgactcagccccactctgtgtcggagtctccggggaagacggtaaccatctcctgcacccgcagcagtggctctatcgaagataagtatgtgcagtggtaccagcagcgcccgggcagttcccccaccattgtgatctattatgataacgaaagaccctctggggtccctgatcggttctctggctccatcgacagctcctccaactctgcctccctcaccatctctggactgaagactgaggacgaggctgactactactgtcagacctacgacaacagcctgtatggttgggtgttcggcggagggaccaagctgaccgtcctaggtcagcccaaggctgccccctcggtcactctgttcccgccctcctctgaggagcttcaagccaacaaggccacactggtgtgtctcataagtgacttctacccgggagccgtgacagtggcttggaaagcagatagcagccccgtcaaggcgggagtggagaccaccacaccctccaaacaaagcaacaacaagtacgcggccagcagctatctgagcctgacgcctgagcagtggaagtcccacagaagctacagctgccaggtcacgcatgaagggagcaccgtggagaagacagtggcccctacagaatgttcataa

SEQ ID NO: 104 - protein, 218 aa, synthetic construct
  REGION 1..218: note = anti-CD19 B11 lambda light chain
NFMLTQPHSVSESPGKTVTISCTRSSGSIEDKYVQWYQQRPGSSPTIVIYYDNERPSGVPDRFSGSIDSSSNSASLTISGLKTEDEADYYCQTYDNSLYGWVFGGGTKLTVLGQPKAAPSVTLFPPSSEELQANKATLVCLISDFYPGAVTVAWKADSSPVKAGVETTTPSKQSNNKYAASSYLSLTPEQWKSHRSYSCQVTHEGSTVEKTVAPTECS

SEQ ID NO: 105 - DNA, 657 bp, synthetic construct
  misc_feature 1..657: note = anti-CD19 D11 lambda light chain
  source 1..657: mol_type = other DNA
aattttatgctgactcagccccactctgtgtcggagtctccggggaagacggtaaccatctcctgcacccgcagcagtggcagcatcgatgataagtttgtgcagtggtaccagcagcgcccgggcagttcccccaccactgtgatctattatgataacattagaccctctggggtccctgatcggttctctggctccatcgacagctcctccaactctgcctccctcaccatctctggactgaagactgaggacgaggctgactactactgtcagtcctatgacgcgagcctgtatggttgggtgttcggcggagggaccaagctgaccgtcctaggtcagcccaaggctgccccctcggtcactctgttcccgccctcctctgaggagcttcaagccaacaaggccacactggtgtgtctcataagtgacttctacccgggagccgtgacagtggcttggaaagcagatagcagccccgtcaaggcgggagtggagaccaccacaccctccaaacaaagcaacaacaagtacgcggccagcagctatctgagcctgacgcctgagcagtggaagtcccacagaagctacagctgccaggtcacgcatgaagggagcaccgtggagaagacagtggcccctacagaatgttcataa

SEQ ID NO: 106 - protein, 218 aa, synthetic construct
  REGION 1..218: note = anti-CD19 D11 lambda light chain
NFMLTQPHSVSESPGKTVTISCTRSSGSIDDKFVQWYQQRPGSSPTTVIYYDNIRPSGVPDRFSGSIDSSSNSASLTISGLKTEDEADYYCQSYDASLYGWVFGGGTKLTVLGQPKAAPSVTLFPPSSEELQANKATLVCLISDFYPGAVTVAWKADSSPVKAGVETTTPSKQSNNKYAASSYLSLTPEQWKSHRSYSCQVTHEGSTVEKTVAPTECS

SEQ ID NO: 107 - DNA, 657 bp, synthetic construct
  misc_feature 1..657: note = anti-CD19 B7 lambda light chain
  source 1..657: mol_type = other DNA
aattttatgctgactcagccccactctgtgtcggagtctccggggaagacggtaaccatctcctgcacccgcagcagtggctctatcgcggataagtatgtgcagtggtaccagcagcgcccgggcagttcccccaccactgtgatctatgaggataaccaaagaccctctggggtccctgatcggttctctggctccatcgacagctcctccaactctgcctccctcaccatctctggactgaagactgaggacgaggctgactactactgtcagtcctatgacagcagcctgtatggttgggtgttcggcggagggaccaagctgaccgtcctaggtcagcccaaggctgccccctcggtcactctgttcccgccctcctctgaggagcttcaagccaacaaggccacactggtgtgtctcataagtgacttctacccgggagccgtgacagtggcttggaaagcagatagcagccccgtcaaggcgggagtggagaccaccacaccctccaaacaaagcaacaacaagtacgcggccagcagctatctgagcctgacgcctgagcagtggaagtcccacagaagctacagctgccaggtcacgcatgaagggagcaccgtggagaagacagtggcccctacagaatgttcataa

SEQ ID NO: 108 - protein, 218 aa, synthetic construct
  REGION 1..218: note = anti-CD19 B7 lambda light chain
NFMLTQPHSVSESPGKTVTISCTRSSGSIADKYVQWYQQRPGSSPTTVIYEDNQRPSGVPDRFSGSIDSSSNSASLTISGLKTEDEADYYCQSYDSSLYGWVFGGGTKLTVLGQPKAAPSVTLFPPSSEELQANKATLVCLISDFYPGAVTVAWKADSSPVKAGVETTTPSKQSNNKYAASSYLSLTPEQWKSHRSYSCQVTHEGSTVEKTVAPTECS

SEQ ID NO: 109 - DNA, 651 bp, synthetic construct
  misc_feature 1..651: note = dummy light chain 1
  source 1..651: mol_type = other DNA
cagtctgtgttgacgcagccgccctcagtgtctgcggccccaggacagaaggtcaccatctcctgctctggaagcagctccaatattgagactggttctgtatcctggtaccagcagctcccaggaacagcccccaaactcctcatttatgacaataataagcgaccctcagggattcctgaccgattctctggctccaagtctggcacgtcagccaccctgggcatcaccggactccagactggggacgaggccgattattactgcggaacatgggatgacagcctgcctggatgggtgttcggcggagggaccaagctgaccgtcctaggtcagcccaaggctgccccctcggtcactctgttcccgccctcctctgaggagcttcaagccaacaaggccacactggtgtgtctcataagtgacttctacccgggagccgtgacagtggcttggaaagcagatagcagccccgtcaaggcgggagtggagaccaccacaccctccaaacaaagcaacaacaagtacgcggccagcagctatctgagcctgacgcctgagcagtggaagtcccacagaagctacagctgccaggtcacgcatgaagggagcaccgtggagaagacagtggcccctacagaatgttcataa

SEQ ID NO: 110 - protein, 216 aa, synthetic construct
  REGION 1..216: note = dummy light chain 1
QSVLTQPPSVSAAPGQKVTISCSGSSSNIETGSVSWYQQLPGTAPKLLIYDNNKRPSGIPDRFSGSKSGTSATLGITGLQTGDEADYYCGTWDDSLPGWVFGGGTKLTVLGQPKAAPSVTLFPPSSEELQANKATLVCLISDFYPGAVTVAWKADSSPVKAGVETTTPSKQSNNKYAASSYLSLTPEQWKSHRSYSCQVTHEGSTVEKTVAPTECS

SEQ ID NO: 111 - DNA, 657 bp, synthetic construct
  misc_feature 1..657: note = dummy light chain 2
  source 1..657: mol_type = other DNA
gaaatagtgatgacgcagtctccagccaccctgtctgtgtctccaggggaaagagccaccctctcctgcagggccagtcagacggttaagaataatttagcctggtaccagcagaaacctggccaggctcccaggctcctcatctatggtgcatccaccagggccactggtatcccagccaggttcagtggcagtgggtctgggacagagttcactctcaccatcagcagcctgcagtctgaagattttgcagtttattactgtcagcagtataacaactggttgcccatcaacccctataccttcggccaagggaccaaggtggaaatcaaacgtacggtggctgcaccatctgtcttcatcttcccgccatctgatgagcagttgaaatctggaactgcctctgttgtgtgcctgctgaataacttctatcccagagaggccaaagtacagtggaaggtggataacgccctccaatcgggtaactcccaggagagtgtcacagagcaggacagcaaggacagcacctacagcctcagcagcaccctgacgctgagcaaagcagactacgagaaacacaaagtctacgcctgcgaagtcacccatcagggcctgagctcgcccgtcacaaagagcttcaacaggggagagtgttaa

SEQ ID NO: 112 - protein, 218 aa, synthetic construct
  REGION 1..218: note = dummy light chain 2
EIVMTQSPATLSVSPGERATLSCRASQTVKNNLAWYQQKPGQAPRLLIYGASTRATGIPARFSGSGSGTEFTLTISSLQSEDFAVYYCQQYNNWLPINPYTFGQGTKVEIKRTVAAPSVFIFPPSDEQLKSGTASVVCLLNNFYPREAKVQWKVDNALQSGNSQESVTEQDSKDSTYSLSSTLTLSKADYEKHKVYACEVTHQGLSSPVTKSFNRGEC

SEQ ID NO: 113 - DNA, 348 bp, synthetic construct
  misc_feature 1..348: note = common variable heavy domain
  source 1..348: mol_type = other DNA
gaggtgcagctgttggagtctgggggaggcttggtacagcctggggggtccctgagactctcctgtgcagcctctggattcacctttagcagctatgccatgagctgggtccgccaggctccagggaaggggctggagtgggtctcagctattagtggtagtggtggtagcacatactacgcagactccgtgaagggccggttcaccatctccagagacaattccaagaacacgctgtatctgcaaatgaacagcctgagagccgaggacacggccgtatattactgtgcgaaaagttatggtgcttttgactactggggccagggaaccctggtcacagtctcgagc

SEQ ID NO: 114 - protein, 116 aa, synthetic construct
  REGION 1..116: note = common variable heavy domain
EVQLLESGGGLVQPGGSLRLSCAASGFTFSSYAMSWVRQAPGKGLEWVSAISGSGGSTYYADSVKGRFTISRDNSKNTLYLQMNSLRAEDTAVYYCAKSYGAFDYWGQGTLVTVSS

SEQ ID NO: 115 - DNA, 324 bp, synthetic construct
  misc_feature 1..324: note = anti-CD47 5A3 kappa variable light domain
  source 1..324: mol_type = other DNA
gacatccagatgacccagtctccatcctccctgtctgcatctgtaggagacagagtcaccatcacttgccaggcgagtcaggacattaataagtatttaaattggtatcagcagaaaccagggaaagcccctaagctcctgatctacggtgcatccaggttggaaacaggggtcccatcaaggttcagtggaagtggatctgggacagattttactttcaccatcagcagcctgcagcctgaagatattgcaacatattactgtcagcagaagcacccccgggggccgaggaccttcggccaagggaccaaggtggaaatcaaa

SEQ ID NO: 116 - protein, 108 aa, synthetic construct
  REGION 1..108: note = anti-CD47 5A3 kappa variable light domain
DIQMTQSPSSLSASVGDRVTITCQASQDINKYLNWYQQKPGKAPKLLIYGASRLETGVPSRFSGSGSGTDFTFTISSLQPEDIATYYCQQKHPRGPRTFGQGTKVEIK

SEQ ID NO: 117 - DNA, 324 bp, synthetic construct
  misc_feature 1..324: note = anti-CD47 5A3-M4 kappa variable light domain
  source 1..324: mol_type = other DNA
gacatccagatgacccagtctccatcctccctgtctgcatctgtaggagacagagtcaccatcacttgccaggcgagtcaggacattaataagtatttaaattggtatcagcagaaaccagggaaagcccctaagctcctgatctacggtgcatccaggttggaaacaggggtcccatcaaggttcagtggaagtggatctgggacagattttactttcaccatcagcagcctgcagcctgaagatattgcaacatattactgtcagcagaagcacccccggaacccgaggaccttcggccaagggaccaaggtggaaatcaaa

SEQ ID NO: 118 - protein, 108 aa, synthetic construct
  REGION 1..108: note = anti-CD47 5A3-M4 kappa variable light domain
DIQMTQSPSSLSASVGDRVTITCQASQDINKYLNWYQQKPGKAPKLLIYGASRLETGVPSRFSGSGSGTDFTFTISSLQPEDIATYYCQQKHPRNPRTFGQGTKVEIK

SEQ ID NO: 119 - DNA, 324 bp, synthetic construct
  misc_feature 1..324: note = anti-CD47 5A3-M3 kappa variable light domain
  source 1..324: mol_type = other DNA
gacatccagatgacccagtctccatcctccctgtctgcatctgtaggagacagagtcaccatcacttgccaggcgagtcagtccattagtagttatttaaattggtatcagcagaaaccagggaaagcccctaagctcctgatctacgctgcatcctcgttggaaacaggggtcccatcaaggttcagtggaagtggatctgggacagattttactttcaccatcagcagcctgcagcctgaagatattgcaacatattactgtcagcagaagcacccccgggggccgaggaccttcggccaagggaccaaggtggaaatcaaa

SEQ ID NO: 120 - protein, 108 aa, synthetic construct
  REGION 1..108: note = anti-CD47 5A3-M3 kappa variable light domain
DIQMTQSPSSLSASVGDRVTITCQASQSISSYLNWYQQKPGKAPKLLIYAASSLETGVPSRFSGSGSGTDFTFTISSLQPEDIATYYCQQKHPRGPRTFGQGTKVEIK

SEQ ID NO: 121 - DNA, 324 bp, synthetic construct
  misc_feature 1..324: note = anti-CD47 5A3-M5 kappa variable light domain
  source 1..324: mol_type = other DNA
gacatccagatgacccagtctccatcctccctgtctgcatctgtaggagacagagtcaccatcacttgccaggcgagtcaggacattaataagtatttaaattggtatcagcagaaaccagggaaagcccctaagctcctgatctacggtgcatccaggttggaaacaggggtcccatcaaggttcagtggaagtggatctgggacagattttactttcaccatcagcagcctgcagcctgaagatattgcaacatattactgtcagcagaagcacccccggtacccgaggaccttcggccaagggaccaaggtggaaatcaaa

SEQ ID NO: 122 - protein, 108 aa, synthetic construct
  REGION 1..108: note = anti-CD47 5A3-M5 kappa variable light domain
DIQMTQSPSSLSASVGDRVTITCQASQDINKYLNWYQQKPGKAPKLLIYGASRLETGVPSRFSGSGSGTDFTFTISSLQPEDIATYYCQQKHPRYPRTFGQGTKVEIK

SEQ ID NO: 123 - DNA, 324 bp, synthetic construct
  misc_feature 1..324: note = anti-CD47 Ke8 kappa variable light domain
  source 1..324: mol_type = other DNA
gacatccagatgacccagtctccatcctccctgtctgcatctgtaggagacagagtcaccatcacttgccgggcaagtcagagcattagcagctatttaaattggtatcagcagaaaccagggaaagcccctaagctcctgatctatgctgcatccagtttgcaaagtggggtcccatcaaggttcagtggcagtggatctgggacagatttcactctcaccatcagcagtctgcaacctgaagattttgcaacttactactgtcagcagttccacaagcggcggccgcagaccttcggccaagggaccaaggtggaaatcaaa

SEQ ID NO: 124 - protein, 108 aa, synthetic construct
  REGION 1..108: note = anti-CD47 Ke8 kappa variable light domain
DIQMTQSPSSLSASVGDRVTITCRASQSISSYLNWYQQKPGKAPKLLIYAASSLQSGVPSRFSGSGSGTDFTLTISSLQPEDFATYYCQQFHKRRPQTFGQGTKVEIK

SEQ ID NO: 125 - DNA, 324 bp, synthetic construct
  misc_feature 1..324: note = anti-CD47 Ke8H5 kappa variable light domain
  source 1..324: mol_type = other DNA
gacatccagatgacccagtctccatcctccctgtctgcatctgtaggagacagagtcaccatcacttgccgggcaagtcagagcattgcgaggtatttaaattggtatcagcagaaaccagggaaagcccctaagctcctgatctatgctgcatccagtttgcaaagtggggtcccatcaaggttcagtggcagtggatctgggacagatttcactctcaccatcagcagtctgcaacctgaagattttgcaacttactactgtcagcagttccataagcgtgcgccgcagaccttcggccaagggaccaaggtggaaatcaaa

SEQ ID NO: 126 - protein, 108 aa, synthetic construct
  REGION 1..108: note = anti-CD47 Ke8H5 kappa variable light domain
DIQMTQSPSSLSASVGDRVTITCRASQSIARYLNWYQQKPGKAPKLLIYAASSLQSGVPSRFSGSGSGTDFTLTISSLQPEDFATYYCQQFHKRAPQTFGQGTKVEIK

SEQ ID NO: 127 - DNA, 324 bp, synthetic construct
  misc_feature 1..324: note = anti-CD47 Ke8B2 kappa variable light domain
  source 1..324: mol_type = other DNA
gacatccagatgacccagtctccatcctccctgtctgcatctgtaggagacagagtcaccatcacttgccgggcaagtcagagcattggtaagtatttaaattggtatcagcagaaaccagggaaagcccctaagctcctgatctatgcggcatccaggttgcaaagtggggtcccatcaaggttcagtggcagtggatctgggacagatttcactctcaccatcagcagtctgcaacctgaagattttgcaacttactactgtcagcagaagcacccgcgtgccccgcggaccttcggccaagggaccaaggtggaaatcaaa

SEQ ID NO: 128 - protein, 108 aa, synthetic construct
  REGION 1..108: note = anti-CD47 Ke8B2 kappa variable light domain
DIQMTQSPSSLSASVGDRVTITCRASQSIGKYLNWYQQKPGKAPKLLIYAASRLQSGVPSRFSGSGSGTDFTLTISSLQPEDFATYYCQQKHPRAPRTFGQGTKVEIK

SEQ ID NO: 129 - DNA, 324 bp, synthetic construct
  misc_feature 1..324: note = anti-CD47 Ke8A2 kappa variable light domain
  source 1..324: mol_type = other DNA
gacatccagatgacccagtctccatcctccctgtctgcatctgtaggagacagagtcaccatcacttgccgggcaagtcagagcattgataggtatttaaattggtatcagcagaaaccagggaaagcccctaagctcctgatctatgctgcatccagtttgcaaagtggggtcccatcaaggttcagtggcagtggatctgggacagatttcactctcaccatcagcagtctgcaacctgaagattttgcaacttactactgtcagcagaagcatccccgtgggccgaggaccttcggccaagggaccaaggtggaaatcaaa

SEQ ID NO: 130 - protein, 108 aa, synthetic construct
  REGION 1..108: note = anti-CD47 Ke8A2 kappa variable light domain
DIQMTQSPSSLSASVGDRVTITCRASQSIDRYLNWYQQKPGKAPKLLIYAASSLQSGVPSRFSGSGSGTDFTLTISSLQPEDFATYYCQQKHPRGPRTFGQGTKVEIK

SEQ ID NO: 131 - DNA, 324 bp, synthetic construct
  misc_feature 1..324: note = anti-CD47 Ke8E8 kappa variable light domain
  source 1..324: mol_type = other DNA
gacatccagatgacccagtctccatcctccctgtctgcatctgtaggagacagagtcaccatcacttgccaggcgagtcaggacattaataagtatttaaattggtatcagcagaaaccagggaaagcccctaagctcctgatctatgctgcatccagtttgcaaagtggggtcccatcaaggttcagtggcagtggatctgggacagatttcactctcaccatcagcagtctgcaacctgaagattttgcaacttactactgtcagcagaagcatccccgtggcccgcggaccttcggccaagggaccaaggtggaaatcaaa

SEQ ID NO: 132 - protein, 108 aa, synthetic construct
  REGION 1..108: note = anti-CD47 Ke8E8 kappa variable light domain
DIQMTQSPSSLSASVGDRVTITCQASQDINKYLNWYQQKPGKAPKLLIYAASSLQSGVPSRFSGSGSGTDFTLTISSLQPEDFATYYCQQKHPRGPRTFGQGTKVEIK

SEQ ID NO: 133 - DNA, 324 bp, synthetic construct
  misc_feature 1..324: note = anti-CD47 Ke8H3 kappa variable light domain
  source 1..324: mol_type = other DNA
gacatccagatgacccagtctccatcctccctgtctgcatctgtaggagacagagtcaccatcacttgccgggcaagtcagagcattaataggtatttaaattggtatcagcagaaaccagggaaagcccctaagctcctgatctatgctgcatccaggttgcaaagtggggtcccatcaaggttcagtggcagtggatctgggacagatttcactctcaccatcagcagtctgcaacctgaagattttgcaacttactactgtcagcagaagcatccgcgtgggccgaggaccttcggccaagggaccaaggtggaaatcaaa

SEQ ID NO: 134 - protein, 108 aa, synthetic construct
  REGION 1..108: note = anti-CD47 Ke8H3 kappa variable light domain
DIQMTQSPSSLSASVGDRVTITCRASQSINRYLNWYQQKPGKAPKLLIYAASRLQSGVPSRFSGSGSGTDFTLTISSLQPEDFATYYCQQKHPRGPRTFGQGTKVEIK

SEQ ID NO: 135 - DNA, 324 bp, synthetic construct
  misc_feature 1..324: note = anti-CD47 Ke8G6 kappa variable light domain
  source 1..324: mol_type = other DNA
gacatccagatgacccagtctccatcctccctgtctgcatctgtaggagacagagtcaccatcacttgccgggcaagtcagagcattggtaggtatttaaattggtatcagcagaaaccagggaaagcccctaagctcctgatctatgctgcatccagtttgcaaagtggggtcccatcaaggttcagtggcagtggatctgggacagatttcactctcaccatcagcagtctgcaacctgaagattttgcaacttactactgtcagcagatgcatccgcgtgcgccgaagaccttcggccaagggaccaaggtggaaatcaaa

SEQ ID NO: 136 - protein, 108 aa, synthetic construct
  REGION 1..108: note = anti-CD47 Ke8G6 kappa variable light domain
DIQMTQSPSSLSASVGDRVTITCRASQSIGRYLNWYQQKPGKAPKLLIYAASSLQSGVPSRFSGSGSGTDFTLTISSLQPEDFATYYCQQMHPRAPKTFGQGTKVEIK

SEQ ID NO: 137 - DNA, 324 bp, synthetic construct
  misc_feature 1..324: note = anti-CD47 Ke8A3 kappa variable light domain
  source 1..324: mol_type = other DNA
gacatccagatgacccagtctccatcctccctgtctgcatctgtaggagacagagtcaccatcacttgccgggtaagtcagagcattagtaagtatttaaattggtatcagcagaaaccagggaaagcccctaagctcctgatctatgctgcatccagtttgcaaagtggggtcccatcaaggttcagtggcagtggatctgggacagatttcactctcaccatcagcagtctgcaacctgaagattttgcaacttactactgtcagcagaggcatccccgtgggccgagcaccttcggccaagggaccaaggtggaaatcaaa

SEQ ID NO: 138 - protein, 108 aa, synthetic construct
  REGION 1..108: note = anti-CD47 Ke8A3 kappa variable light domain
DIQMTQSPSSLSASVGDRVTITCRVSQSISKYLNWYQQKPGKAPKLLIYAASSLQSGVPSRFSGSGSGTDFTLTISSLQPEDFATYYCQQRHPRGPSTFGQGTKVEIK

SEQ ID NO: 139 - DNA, 324 bp, synthetic construct
  misc_feature 1..324: note = anti-CD47 Ke81A3 kappa variable light domain
  source 1..324: mol_type = other DNA
gacatccagatgacccagtctccatcctccctgtctgcatctgtaggagacagagtcaccatcacttgccaggcgagtcaggacattaataggtatttaaattggtatcagcagaaaccagggaaagcccctaagctcctgatctatgctgcatccagtttgcaaagtggggtcccatcaaggttcagtggcagtggatctgggacagatttcactctcaccatcagcagtctgcaacctgaagattttgcaacttactactgtcagcagaggcatccgcgtgccccgcggaccttcggccaagggaccaaggtggaaatcaaa

SEQ ID NO: 140 - protein, 108 aa, synthetic construct
  REGION 1..108: note = anti-CD47 Ke81A3 kappa variable light domain
DIQMTQSPSSLSASVGDRVTITCQASQDINRYLNWYQQKPGKAPKLLIYAASSLQSGVPSRFSGSGSGTDFTLTISSLQPEDFATYYCQQRHPRAPRTFGQGTKVEIK

SEQ ID NO: 141 - DNA, 324 bp, synthetic construct
  misc_feature 1..324: note = anti-CD47 Ke8A8 kappa variable light domain
  source 1..324: mol_type = other DNA
gacatccagatgacccagtctccatcctccctgtctgcatctgtaggagacagagtcaccatcacttgccgggcaagtcagagcattagtaagtatttaaattggtatcagcagaaaccagggaaagcccctaagctcctgatctatgctgcatccactttgcaaagtggggtcccatcaaggttcagtggcagtggatctgggacagatttcactctcaccatcagcagtctgcaacctgaagattttgcaacttactactgtcagcagatgcatccgcgtgcgccgaagaccttcggccaagggaccaaggtggaaatcaaa

SEQ ID NO: 142 - protein, 108 aa, synthetic construct
  REGION 1..108: note = anti-CD47 Ke8A8 kappa variable light domain
DIQMTQSPSSLSASVGDRVTITCRASQSISKYLNWYQQKPGKAPKLLIYAASTLQSGVPSRFSGSGSGTDFTLTISSLQPEDFATYYCQQMHPRAPKTFGQGTKVEIK

SEQ ID NO: 143 - DNA, 324 bp, synthetic construct
  misc_feature 1..324: note = anti-CD47 Ke8C7 kappa variable light domain
  source 1..324: mol_type = other DNA
gacatccagatgacccagtctccatcctccctgtctgcatctgtaggagacagagtcaccatcacttgccaggcgagtcaggacattaataggtatttaaattggtatcagcagaaaccagggaaagcccctaagctcctgatctatgctgcatccagtttgcaaagtggggtcccatcaaggttcagtggcagtggatctgggacagatttcactctcaccatcagcagtctgcaacctgaagattttgcaacttactactgtcagcagcgccatccgcgtggcccgaggaccttcggccaagggaccaaggtggaaatcaaa

SEQ ID NO: 144 - protein, 108 aa, synthetic construct
  REGION 1..108: note = anti-CD47 Ke8C7 kappa variable light domain
DIQMTQSPSSLSASVGDRVTITCQASQDINRYLNWYQQKPGKAPKLLIYAASSLQSGVPSRFSGSGSGTDFTLTISSLQPEDFATYYCQQRHPRGPRTFGQGTKVEIK

SEQ ID NO: 145 - DNA, 324 bp, synthetic construct
  misc_feature 1..324: note = anti-CD47 Ke8G2 kappa variable light domain
  source 1..324: mol_type = other DNA
gacatccagatgacccagtctccatcctccctgtctgcatctgtaggagacagagtcaccatcacttgccgggcaagtcagagcattggtaggtatttaaattggtatcagcagaaaccagggaaagcccctaagctcctgatctatgcggcatccaggttgcaaagtggggtcccatcaaggttcagtggcagtggatctgggacagatttcactctcaccatcaacagtctgcaacctgaagattttgcaacttactactgtcagcagaagcatccccgtgcgccgaggaccttcggccaagggaccaaggtggaaatcaaa

SEQ ID NO: 146 - protein, 108 aa, synthetic construct
  REGION 1..108: note = anti-CD47 Ke8G2 kappa variable light domain
DIQMTQSPSSLSASVGDRVTITCRASQSIGRYLNWYQQKPGKAPKLLIYAASRLQSGVPSRFSGSGSGTDFTLTINSLQPEDFATYYCQQKHPRAPRTFGQGTKVEIK

SEQ ID NO: 147 - DNA, 324 bp, synthetic construct
  misc_feature 1..324: note = anti-CD47 Ke81G9 kappa variable light domain
  source 1..324: mol_type = other DNA
gacatccagatgacccagtctccatcctccctgtctgcatctgtaggagacagagtcaccatcacttgccgggcaagtcagagcattgataagtatttaaattggtatcagcagaaaccagggaaagcccctaagctcctgatctatgcggcatccaggttgcaaagtggggtcccatcaaggttcagtggcagtggatctgggacagatttcactctcaccatcagcagtctgcaacctgaagattttgcaacttactactgtcagcagcggcataagcgttccccgcagaccttcggccaagggaccaaggtggaaatcaaa

SEQ ID NO: 148 - protein, 108 aa, synthetic construct
  REGION 1..108: note = anti-CD47 Ke81G9 kappa variable light domain
DIQMTQSPSSLSASVGDRVTITCRASQSIDKYLNWYQQKPGKAPKLLIYAASRLQSGVPSRFSGSGSGTDFTLTISSLQPEDFATYYCQQRHKRSPQTFGQGTKVEIK

SEQ ID NO: 149 - DNA, 324 bp, synthetic construct
  misc_feature 1..324: note = anti-CD47 Ke8F2 kappa variable light domain
  source 1..324: mol_type = other DNA
gacatccagatgacccagtctccatcctccctgtctgcatctgtaggagacagagtcaccatcacttgccgggcaagtcagagcattgataagtatttaaattggtatcagcagaaaccagggaaagcccctaagctcctgatctatgctgcatccagtttgcaaagtggggtcccatcaaggttcagtggcagtggatctgggacagatttcactctcaccatcagcagtctgcaacctgaagattttgcaacttactactgtcagcagaagcatccgcgtgcgccgcggaccttcggccaagggaccaaggtggaaatcaaa

SEQ ID NO: 150 - protein, 108 aa, synthetic construct
  REGION 1..108: note = anti-CD47 Ke8F2 kappa variable light domain
DIQMTQSPSSLSASVGDRVTITCRASQSIDKYLNWYQQKPGKAPKLLIYAASSLQSGVPSRFSGSGSGTDFTLTISSLQPEDFATYYCQQKHPRAPRTFGQGTKVEIK

SEQ ID NO: 151 - DNA, 324 bp, synthetic construct
  misc_feature 1..324: note = anti-CD47 Ke8B7 kappa variable light domain
  source 1..324: mol_type = other DNA
gacatccagatgacccagtctccatcctccctgtctgcatctgtaggagacagagtcaccatcacttgccgggcaagtcagagcattgggaagtatttaaattggtatcagcagaaaccagggaaagcccctaagctcctgatctatgctgcatccagtttgcaaagtggggtcccatcaaggttcagtggcagtggatctgggacagatttcactctcaccatcagcagtctgcaacctgaagattttgcaacttactactgtcagcagatgcatccgcgtagcccgaagaccttcggccaagggaccaaggtggaaatcaaa

SEQ ID NO: 152 - protein, 108 aa, synthetic construct
  REGION 1..108: note = anti-CD47 Ke8B7 kappa variable light domain
DIQMTQSPSSLSASVGDRVTITCRASQSIGKYLNWYQQKPGKAPKLLIYAASSLQSGVPSRFSGSGSGTDFTLTISSLQPEDFATYYCQQMHPRSPKTFGQGTKVEIK

SEQ ID NO: 153 - DNA, 324 bp, synthetic construct
  misc_feature 1..324: note = anti-CD47 Ke8C4 kappa variable light domain
  source 1..324: mol_type = other DNA
gacatccagatgacccagtctccatcctccctgtctgcatctgtaggagacagagtcaccatcacttgccgggcaagtcagagcattagtaggtatttaaattggtatcagcagaaaccagggaaagcccctaagctcctgatctatgctgcatccaatttgcaaagtggggtcccatcaaggttcagtggcagtggatctgggacagatttcactctcaccatcagcagtctgcaacctgaagattttgcaacttactactgtcagcagatgcatccgcgtgggccgaagaccttcggccaagggaccaaggtggaaatcaaa

SEQ ID NO: 154 - protein, 108 aa, synthetic construct
  REGION 1..108: note = anti-CD47 Ke8C4 kappa variable light domain
DIQMTQSPSSLSASVGDRVTITCRASQSISRYLNWYQQKPGKAPKLLIYAASNLQSGVPSRFSGSGSGTDFTLTISSLQPEDFATYYCQQMHPRGPKTFGQGTKVEIK

SEQ ID NO: 155 - DNA, 324 bp, synthetic construct
  misc_feature 1..324: note = anti-CD47 Ke8F1 kappa variable light domain
  source 1..324: mol_type = other DNA
gacatccagatgacccagtctccatcctccctgtctgcatctgtaggagacagagtcaccatcacttgccgggcaagtcagagcattgcttcttatgtaaattggtatcagcagaaaccagggaaagcccctaagctcctgatctatgctgcatccggtttgcaaagtggggtcccatcaaggttcagtggcagtggatctgggacagatttcactctcaccatcagcagtctgcaacctgaagattttgcaacttactactgtcagcagttccataagcgtcggccgcagaccttcggccaagggaccaaggtggaaatcaaa

SEQ ID NO: 156 - protein, 108 aa, synthetic construct
  REGION 1..108: note = anti-CD47 Ke8F1 kappa variable light domain
DIQMTQSPSSLSASVGDRVTITCRASQSIASYVNWYQQKPGKAPKLLIYAASGLQSGVPSRFSGSGSGTDFTLTISSLQPEDFATYYCQQFHKRRPQTFGQGTKVEIK

SEQ ID NO: 157 - DNA, 324 bp, synthetic construct
  misc_feature 1..324: note = anti-CD47 Ke8G11 kappa variable light domain
  source 1..324: mol_type = other DNA
gacatccagatgacccagtctccatcctccctgtctgcatctgtaggagacagagtcaccatcacttgccgggcaagtcagagcattgggaggtatttaaattggtatcagcagaaaccagggaaagcccctaagctcctgatctatgctgcatccagtttgcaaagtggggtcccatcaaggttcagtggcagtggatctgggacagatttcactctcaccatcagcagtctgcaacctgaagattttgcaacttactactgtcagcagatgcatccgcgtgggccgaagaccttcggccaagggaccaaggtggaaatcaaa

SEQ ID NO: 158 - protein, 108 aa, synthetic construct
  REGION 1..108: note = anti-CD47 Ke8G11 kappa variable light domain
DIQMTQSPSSLSASVGDRVTITCRASQSIGRYLNWYQQKPGKAPKLLIYAASSLQSGVPSRFSGSGSGTDFTLTISSLQPEDFATYYCQQMHPRGPKTFGQGTKVEIK

SEQ ID NO: 159 - DNA, 324 bp, synthetic construct
  misc_feature 1..324: note = anti-CD47 Ke8H6 kappa variable light domain
  source 1..324: mol_type = other DNA
gacatccagatgacccagtctccatcctccctgtctgcatctgtaggagacagagtcaccatcacttgccgggcaagtcagagcattagtaagtatttaaattggtatcagcagaaaccagggaaagcccctaagctcctgatctataatgcatccactttgcaaagtggggtcccatcaaggttcagtggcagtggatctgggacagatttcactctcaccatcagcagtctgcaacctgaagattttgcaacttactactgtcagcagaggcatccgcgtgggccgcgcaccttcggccaagggaccaaggtggaaatcaaa

SEQ ID NO: 160 - protein, 108 aa, synthetic construct
  REGION 1..108: note = anti-CD47 Ke8H6 kappa variable light domain
DIQMTQSPSSLSASVGDRVTITCRASQSISKYLNWYQQKPGKAPKLLIYNASTLQSGVPSRFSGSGSGTDFTLTISSLQPEDFATYYCQQRHPRGPRTFGQGTKVEIK

SEQ ID NO: 161 - DNA, 324 bp, synthetic construct
  misc_feature 1..324: note = anti-CD47 Ke84G9 kappa variable light domain
  source 1..324: mol_type = other DNA
gacatccagatgacccagtctccatcctccctgtctgcatctgtaggagacagagtcaccatcacttgccgggcaagtcagagcattagtaagtatttaaattggtatcagcagaaaccagggaaagcccctaagctcctgatctatgctgcatccagtttgcaaagtggggtcccatcaaggttcagtggcagtggatctgggacagatttcactctcaccatcagcagtctgcaacctgaagattttgcaacttactactgtcagcagaagcatccgcgtagcccgcggaccttcggccaagggaccaaggtggaaatcaaa

SEQ ID NO: 162 - protein, 108 aa, synthetic construct
  REGION 1..108: note = anti-CD47 Ke84G9 kappa variable light domain
DIQMTQSPSSLSASVGDRVTITCRASQSISKYLNWYQQKPGKAPKLLIYAASSLQSGVPSRFSGSGSGTDFTLTISSLQPEDFATYYCQQKHPRSPRTFGQGTKVEIK

SEQ ID NO: 163 - DNA, 324 bp, synthetic construct
  misc_feature 1..324: note = anti-CD47 Ke8A4 kappa variable light domain
  source 1..324: mol_type = other DNA
gacatccagatgacccagtctccatcctccctgtctgcatctgtaggagacagagtcaccatcacttgccgggcaagtcagagcattgctaagtatttaaattggtatcagcagaaaccagggaaagcccctaagctcctgatctatgctgcatccagtttgcaaagtggggtcccatcaaggttcagtggcagtggatctgggacagatttcactctcaccatcagcagtctgcaacctgaagattttgcaacttactactgtcagcagttccataagcgtagcccgcagaccttcggccaagggaccaaggtggaaatcaaa

SEQ ID NO: 164 - protein, 108 aa, synthetic construct
  REGION 1..108: note = anti-CD47 Ke8A4 kappa variable light domain
DIQMTQSPSSLSASVGDRVTITCRASQSIAKYLNWYQQKPGKAPKLLIYAASSLQSGVPSRFSGSGSGTDFTLTISSLQPEDFATYYCQQFHKRSPQTFGQGTKVEIK

SEQ ID NO: 165 - DNA, 324 bp, synthetic construct
  misc_feature 1..324: note = anti-CD47 Ke86G9 kappa variable light domain
  source 1..324: mol_type = other DNA
gacatccagatgacccagtctccatcctccctgtctgcatctgtaggagacagagtcaccatcacttgccgggcaagtcagagcattagtaagtatttaaattggtatcagcagaaaccagggaaagcccctaagctcctgatctataatgcatccaatttgcaaagtggggtcccatcaaggttcagtggcagtggatctgggacagatttcactctcaccatcagcagtctgcaacctgaagattttgcaacttactactgtcagcagaggcatccgcgtgggccgaccaccttcggccaagggaccaaggtggaaatcaaa

SEQ ID NO: 166 - protein, 108 aa, synthetic construct
  REGION 1..108: note = anti-CD47 Ke86G9 kappa variable light domain
DIQMTQSPSSLSASVGDRVTITCRASQSISKYLNWYQQKPGKAPKLLIYNASNLQSGVPSRFSGSGSGTDFTLTISSLQPEDFATYYCQQRHPRGPTTFGQGTKVEIK

SEQ ID NO: 167 - DNA, 324 bp, synthetic construct
  misc_feature 1..324: note = anti-CD47 Ka3 kappa variable light domain
  source 1..324: mol_type = other DNA
gacatccagatgacccagtctccatcctccctgtctgcatctgtaggagacagagtcaccatcacttgccgggcaagtcagagcattagcagctatttaaattggtatcagcagaaaccagggaaagcccctaagctcctgatctatgctgcatccagtttgcaaagtggggtcccatcaaggttcagtggcagtggatctgggacagatttcactctcaccatcagcagtctgcaacctgaagattttgcaacttactactgtcagcagatgcacccgcgcgccccgaagaccttcggccaagggaccaaggtggaaatcaaa

SEQ ID NO: 168 - protein, 108 aa, synthetic construct
  REGION 1..108: note = anti-CD47 Ka3 kappa variable light domain
DIQMTQSPSSLSASVGDRVTITCRASQSISSYLNWYQQKPGKAPKLLIYAASSLQSGVPSRFSGSGSGTDFTLTISSLQPEDFATYYCQQMHPRAPKTFGQGTKVEIK

SEQ ID NO: 169 - DNA, 324 bp, synthetic construct
  misc_feature 1..324: note = anti-CD47 Ka3A2 kappa variable light domain
  source 1..324: mol_type = other DNA
gacatccagatgacccagtctccatcctccctgtctgcatctgtaggagacagagtcaccatcacttgccgggcaagtcagagcattagtaagtatttaaattggtatcagcagaaaccagggaaagcccctaagctcctgatctatgctgcatccaggttgcaaagtggggtcccatcaaggttcagtggcagtggatctgggacagatttcactctcaccatcagcagtctgcaacctgaagattttgcaacttactactgtcagcagatgcatcctcgctcgccgaaaaccttcggccaagggaccaaggtggaaatcaaa

SEQ ID NO: 170 - protein, 108 aa, synthetic construct
  REGION 1..108: note = anti-CD47 Ka3A2 kappa variable light domain
DIQMTQSPSSLSASVGDRVTITCRASQSISKYLNWYQQKPGKAPKLLIYAASRLQSGVPSRFSGSGSGTDFTLTISSLQPEDFATYYCQQMHPRSPKTFGQGTKVEIK

SEQ ID NO: 171 - DNA, 324 bp, synthetic construct
  misc_feature 1..324: note = anti-CD47 Ka3H3 kappa variable light domain
  source 1..324: mol_type = other DNA
gacatccagatgacccagtctccatcctccctgtctgcatctgtaggagacagagtcaccatcacttgccaggcgagtcaggacattgctaagtatttaaattggtatcagcagaaaccagggaaagcccctaagctcctgatctatgctgcatccgctttgcaaagtggggtcccatcaaggttcagtggcagtggatctgggacagatttcactctcaccatcagcagtctgcaacctgaagattttgcaacttactactgtcagcagatgcatcctcgctcgccgaaaaccttcggccaagggaccaaggtggaaatcaaa

SEQ ID NO: 172 - protein, 108 aa, synthetic construct
  REGION 1..108: note = anti-CD47 Ka3H3 kappa variable light domain
DIQMTQSPSSLSASVGDRVTITCQASQDIAKYLNWYQQKPGKAPKLLIYAASALQSGVPSRFSGSGSGTDFTLTISSLQPEDFATYYCQQMHPRSPKTFGQGTKVEIK

SEQ ID NO: 173 - DNA, 324 bp, synthetic construct
  misc_feature 1..324: note = anti-CD47 Ka3A3 kappa variable light domain
  source 1..324: mol_type = other DNA
gacatccagatgacccagtctccatcctccctgtctgcatctgtaggagacagagtcaccatcacttgccgggcaagtcagagcattgctagttatttaaattggtatcagcagaaaccagggaaagcccctaagctcctgatctatgcggcatccaggttgcaaagtggggtcccatcaaggttcagtggcagtggatctgggacagatttcactctcaccatcagcagtctgcaacctgaagattttgcaacttactactgtcagcagatgcatcctcgcgcgccgaaaaccttcggccaagggaccaaggtggaaatcaaa

SEQ ID NO: 174 - protein, 108 aa, synthetic construct
  REGION 1..108: note = anti-CD47 Ka3A3 kappa variable light domain
DIQMTQSPSSLSASVGDRVTITCRASQSIASYLNWYQQKPGKAPKLLIYAASRLQSGVPSRFSGSGSGTDFTLTISSLQPEDFATYYCQQMHPRAPKTFGQGTKVEIK

SEQ ID NO: 175 - DNA, 324 bp, synthetic construct
  misc_feature 1..324: note = anti-CD47 Ka3H8 kappa variable light domain
  source 1..324: mol_type = other DNA
gacatccagatgacccagtctccatcctccctgtctgcatctgtaggagacagagtcaccatcacttgccgggcaagtcagagcattgcgagttatttaaattggtatcagcagaaaccagggaaagcccctaagctcctgatctatgcggcatccaggttgcaaagtggggtcccatcaaggttcagtggcagtggatctgggacagatttcactctcaccatcagcagtctgcaacctgaagattttgcaacttactactgtcagcagatgcatcctcgctcgccgaaaaccttcggccaagggaccaaggtggaaatcaaa

SEQ ID NO: 176 - protein, 108 aa, synthetic construct
  REGION 1..108: note = anti-CD47 Ka3H8 kappa variable light domain
DIQMTQSPSSLSASVGDRVTITCRASQSIASYLNWYQQKPGKAPKLLIYAASRLQSGVPSRFSGSGSGTDFTLTISSLQPEDFATYYCQQMHPRSPKTFGQGTKVEIK

SEQ ID NO: 177 - DNA, 324 bp, synthetic construct
  misc_feature 1..324: note = anti-CD47 Ka3B2 kappa variable light domain
  source 1..324: mol_type = other DNA
gacatccagatgacccagtctccatcctccctgtctgcatctgtaggagacagagtcaccatcacttgccgggcaagtcagaacattggtaagtatttaaattggtatcagcagaaaccagggaaagcccctaagctcctgatctatagtgcatccaggttgcaaagtggggtcccatcaaggttcagtggcagtggatctgggacagatttcactctcaccatcagcagtctgcaacctgaagattttgcaacttactactgtcagcagatgcatcctcgcgcgccgaaaaccttcggccaagggaccaaggtggaaatcaaa

SEQ ID NO: 178 - protein, 108 aa, synthetic construct
  REGION 1..108: note = anti-CD47 Ka3B2 kappa variable light domain
DIQMTQSPSSLSASVGDRVTITCRASQNIGKYLNWYQQKPGKAPKLLIYSASRLQSGVPSRFSGSGSGTDFTLTISSLQPEDFATYYCQQMHPRAPKTFGQGTKVEIK

SEQ ID NO: 179 - DNA, 324 bp, synthetic construct
  misc_feature 1..324: note = anti-CD47 Ka3C5 kappa variable light domain
  source 1..324: mol_type = other DNA
gacatccagatgacccagtctccatcctccctgtctgcatctgtaggagacagagtcaccatcacttgccgggcaagtcagagcattagtaggtatttaaattggtatcagcagaaaccagggaaagcccctaagctcctgatctattctgcatcctctttgcaaagtggggtcccatcaaggttcagtggcagtggatctgggacagatttcactctcaccatcagcagtctgcaacctgaagattttgcaacttactactgtcagcagatgcatcctcgcgccccgaaaaccttcggccaagggaccaaggtggaaatcaaa

SEQ ID NO: 180 - protein, 108 aa, synthetic construct
  REGION 1..108: note = anti-CD47 Ka3C5 kappa variable light domain
DIQMTQSPSSLSASVGDRVTITCRASQSISRYLNWYQQKPGKAPKLLIYSASSLQSGVPSRFSGSGSGTDFTLTISSLQPEDFATYYCQQMHPRAPKTFGQGTKVEIK

SEQ ID NO: 181 - DNA, 324 bp, synthetic construct
  misc_feature 1..324: note = anti-CD47 Ka3G2 kappa variable light domain
  source 1..324: mol_type = other DNA
gacatccagatgacccagtctccatcctccctgtctgcatctgtaggagacagagtcaccatcacttgccgggcaagtcagagcattgataagtatttaaattggtatcagcagaaaccagggaaagcccctaagctcctgatctatgctgcatccaggttgcaaagtggggtcccatcaaggttcagtggcagtggatctgggacagatttcactctcaccatcagcagtctgcaacctgaagattttgcaacttactactgtcagcagatgcatcctcgcgggccgaaaaccttcggccaagggaccaaggtggaaatcaaa

SEQ ID NO: 182 - protein, 108 aa, synthetic construct
  REGION 1..108: note = anti-CD47 Ka3G2 kappa variable light domain
DIQMTQSPSSLSASVGDRVTITCRASQSIDKYLNWYQQKPGKAPKLLIYAASRLQSGVPSRFSGSGSGTDFTLTISSLQPEDFATYYCQQMHPRGPKTFGQGTKVEIK

SEQ ID NO: 183 - DNA, 324 bp, synthetic construct
  misc_feature 1..324: note = anti-CD47 Ka3D3 kappa variable light domain
  source 1..324: mol_type = other DNA
gacatccagatgacccagtctccatcctccctgtctgcatctgtaggagacagagtcaccatcacttgccgggcaagtcagagcattggtaagtatttaaattggtatcagcagaaaccagggaaagcccctaagctcctgatctatgctgcatccaggttgcaaagtggggtcccatcaaggttcagtggcagtggatctgggacagatttcactctcaccatcagcagtctgcaacctgaagattttgcaacttactactgtcagcagatgcatcctcgcgcgccgaaaaccttcggccaagggaccaaggtggaaatcaaa

SEQ ID NO: 184 - protein, 108 aa, synthetic construct
  REGION 1..108: note = anti-CD47 Ka3D3 kappa variable light domain
DIQMTQSPSSLSASVGDRVTITCRASQSIGKYLNWYQQKPGKAPKLLIYAASRLQSGVPSRFSGSGSGTDFTLTISSLQPEDFATYYCQQMHPRAPKTFGQGTKVEIK

SEQ ID NO: 185 - DNA, 333 bp, synthetic construct
  misc_feature 1..333: note = anti-CD47 Kc4 kappa variable light domain
  source 1..333: mol_type = other DNA
cagtctgccctgactcagcctgcctccgtgtctgggtctcctggacagtcgatcaccatctcctgcactggaaccagcagtgacgttggtggttataactatgtctcctggtaccaacagcacccaggcaaagcccccaaactcatgatttatgaggtcagtaatcggccctcaggggtttctaatcgcttctctggctccaagtctggcaacacggcctccctgaccatctctgggctccaggctgaggacgaggctgattattactgcagctcatatgattggtggttccgccccaaggtgttcggcggagggaccaagctgaccgtccta

SEQ ID NO: 186 - protein, 111 aa, synthetic construct
  REGION 1..111: note = anti-CD47 Kc4 kappa variable light domain
QSALTQPASVSGSPGQSITISCTGTSSDVGGYNYVSWYQQHPGKAPKLMIYEVSNRPSGVSNRFSGSKSGNTASLTISGLQAEDEADYYCSSYDWWFRPKVFGGGTKLTVL

SEQ ID NO: 187 - DNA, 333 bp, synthetic construct
  misc_feature 1..333: note = anti-CD47 Kc4G11 kappa variable light domain
  source 1..333: mol_type = other DNA
cagtctgccctgactcagcctgcctccgtgtctgggtctcctggacagtcgatcaccatctcctgcactggaaccagcagtgacgttgggaaggcgaactatgtctcctggtaccaacagcacccaggcaaagcccccaaactcatgatttataaggatagtgatcggccctcaggggtttctaatcgcttctctggctccaagtctggcaacacggcctccctgaccatctctgggctccaggctgaggacgaggctgattattactgcagctcatatgattggtggttccgccccaaggtgttcggcggagggaccaagctgaccgtccta

SEQ ID NO: 188 - protein, 111 aa, synthetic construct
  REGION 1..111: note = anti-CD47 Kc4G11 kappa variable light domain
QSALTQPASVSGSPGQSITISCTGTSSDVGKANYVSWYQQHPGKAPKLMIYKDSDRPSGVSNRFSGSKSGNTASLTISGLQAEDEADYYCSSYDWWFRPKVFGGGTKLTVL

SEQ ID NO: 189 - DNA, 333 bp, synthetic construct
  misc_feature 1..333: note = anti-CD47 Kc4C11 kappa variable light domain
  source 1..333: mol_type = other DNA
cagtctgccctgactcagcctgcctccgtgtctgggtctcctggacagtcgatcaccatctcctgcactggaaccagcagtgacgttagggggaataactatgtctcctggtaccaacagcacccaggcaaagcccccaaactcatgatttatgagaatagtaagcggccctcaggggtttctaatcgcttctctggctccaagtctggcaacacggcctccctgaccatctctgggctccaggctgaggacgaggctgattattactgcagctcatatgattggtggttccgccccaaggtgttcggcggagggaccaagctgaccgtccta

SEQ ID NO: 190 - protein, 111 aa, synthetic construct
  REGION 1..111: note = anti-CD47 Kc4C11 kappa variable light domain
QSALTQPASVSGSPGQSITISCTGTSSDVRGNNYVSWYQQHPGKAPKLMIYENSKRPSGVSNRFSGSKSGNTASLTISGLQAEDEADYYCSSYDWWFRPKVFGGGTKLTVL

SEQ ID NO: 191 - DNA, 333 bp, synthetic construct
  misc_feature 1..333: note = anti-CD47 Kc4A1 kappa variable light domain
  source 1..333: mol_type = other DNA
cagtctgccctgactcagcctgcctccgtgtctgggtctcctggacagtcgatcaccatctcctgcactggaaccagcagtgacgttagtgcgaggaactatgtctcctggtaccaacagcacccaggcaaagcccccaaactcatgatttatgagagtagtaagcggccctcaggggtttctaatcgcttctctggctccaagtctggcaacacggcctccctgaccatctctgggctccaggctgaggacgaggctgattattactgcagctcatatgattggtggttccgccccaaggtgttcggcggagggaccaagctgaccgtccta

SEQ ID NO: 192 - protein, 111 aa, synthetic construct
  REGION 1..111: note = anti-CD47 Kc4A1 kappa variable light domain
QSALTQPASVSGSPGQSITISCTGTSSDVSARNYVSWYQQHPGKAPKLMIYESSKRPSGVSNRFSGSKSGNTASLTISGLQAEDEADYYCSSYDWWFRPKVFGGGTKLTVL

SEQ ID NO: 193 - DNA, 333 bp, synthetic construct
  misc_feature 1..333: note = anti-CD47 Kc4A4 kappa variable light domain
  source 1..333: mol_type = other DNA
cagtctgccctgactcagcctgcctccgtgtctgggtctcctggacagtcgatcaccatctcctgcactagaaccagcagtgacgttaataatactaactatgtctcctggtaccaacagcacccaggcaaagcccccaaactcatgatttataagactagtggtcggccctcaggggtttctaatcgcttctctggctccaagtctggcaacacggcctccctgaccatctctgggctccaggctgaggacgaggctgattattactgcagctcatatgattggtggttccgccccaaggtgttcggcggagggaccaagctgaccgtccta

SEQ ID NO: 194 - protein, 111 aa, synthetic construct
  REGION 1..111: note = anti-CD47 Kc4A4 kappa variable light domain
QSALTQPASVSGSPGQSITISCTRTSSDVNNTNYVSWYQQHPGKAPKLMIYKTSGRPSGVSNRFSGSKSGNTASLTISGLQAEDEADYYCSSYDWWFRPKVFGGGTKLTVL

SEQ ID NO: 195 - DNA, 333 bp, synthetic construct
  misc_feature 1..333: note = anti-CD47 Kc4E10 kappa variable light domain
  source 1..333: mol_type = other DNA
cagtctgccctgactcagcctgcctccgtgtctgggtctcctggacagtcgatcaccatctcctgcactggaaccagcagtgacgttaattctgctaactatgtctcctggtaccaacagcacccaggcaaagcccccaaactcatgatttataagagtagtagtcggccctcaggggtttctaatcgcttctctggctccaagtctggcaacacggcctccctgaccatctctgggctccaggctgaggacgaggctgattattactgcagctcatatgattggtggttccgccccaaggtgttcggcggagggaccaagctgaccgtccta

SEQ ID NO: 196 - protein, 111 aa, synthetic construct
  REGION 1..111: note = anti-CD47 Kc4E10 kappa variable light domain
QSALTQPASVSGSPGQSITISCTGTSSDVNSANYVSWYQQHPGKAPKLMIYKSSSRPSGVSNRFSGSKSGNTASLTISGLQAEDEADYYCSSYDWWFRPKVFGGGTKLTVL

SEQ ID NO: 197 - DNA, 333 bp, synthetic construct
  misc_feature 1..333: note = anti-CD47 Kc4G9 kappa variable light domain
  source 1..333: mol_type = other DNA
cagtctgccctgactcagcctgcctccgtgtccgggtctcctggacagtcgatcaccatctcctgcactggaaccagcagtgacgttgagaggaagaactatgtctcctggtaccaacagcacccaggcaaagcccccaaactcatgatttataagaatagtactcggccctcaggggtttctaatcgcttctctggctccaagtctggcaacacggcctccctgaccatctctgggctccaggctgaggacgaggctgattattactgcagctcatatgattggtggttccgccccaaggtgttcggcggagggaccaagctgaccgtccta

SEQ ID NO: 198 - protein, 111 aa, synthetic construct
  REGION 1..111: note = anti-CD47 Kc4G9 kappa variable light domain
QSALTQPASVSGSPGQSITISCTGTSSDVERKNYVSWYQQHPGKAPKLMIYKNSTRPSGVSNRFSGSKSGNTASLTISGLQAEDEADYYCSSYDWWFRPKVFGGGTKLTVL

SEQ ID NO: 199 - DNA, 333 bp, synthetic construct
  misc_feature 1..333: note = anti-CD47 Kc4C3 kappa variable light domain
  source 1..333: mol_type = other DNA
cagtctgccctgactcagcctgcctccgtgtctgggtctcctggacagtcgatcaccatctcctgcactggaaccagcagtgacgttagggcggctaactatgtctcctggtaccaacagcacccaggcaaagcccccaaactcatgatttataagaatagtactcggccctcaggggtttctaatcgcttctctggctccaagtctggcaacacggcctccctgaccatctctgggctccaggctgaggacgaggctgattattactgcagctcatatgattggtggttccgccccaaggtgttcggcggagggaccaagctgaccgtccta

SEQ ID NO: 200 - protein, 111 aa, synthetic construct
  REGION 1..111: note = anti-CD47 Kc4C3 kappa variable light domain
QSALTQPASVSGSPGQSITISCTGTSSDVRAANYVSWYQQHPGKAPKLMIYKNSTRPSGVSNRFSGSKSGNTASLTISGLQAEDEADYYCSSYDWWFRPKVFGGGTKLTVL

SEQ ID NO: 201 - DNA, 333 bp, synthetic construct
  misc_feature 1..333: note = anti-CD47 Kc4F4 kappa variable light domain
  source 1..333: mol_type = other DNA
cagtctgccctgactcagcctgcctccgtgtctgggtctcctggacagtcgatcaccatctcctgcactggaaccagcagtgacgttaggagggctaactatgtctcctggtaccaacagcacccaggcaaagcccccaaactcatgatttatcaggatagtagtcggccctcaggggtttctaatcgcttctctggctccaagtctggcaacacggcctccctgaccatctctgggctccaggctgaggacgaggctgattattactgcagctcatatgattggtggttccgccccaaggtgttcggcggagggaccaagctgaccgtccta

SEQ ID NO: 202 - protein, 111 aa, synthetic construct
  REGION 1..111: note = anti-CD47 Kc4F4 kappa variable light domain
QSALTQPASVSGSPGQSITISCTGTSSDVRRANYVSWYQQHPGKAPKLMIYQDSSRPSGVSNRFSGSKSGNTASLTISGLQAEDEADYYCSSYDWWFRPKVFGGGTKLTVL

SEQ ID NO: 203 - DNA, 333 bp, synthetic construct
  misc_feature 1..333: note = anti-CD47 Kc4B1 kappa variable light domain
  source 1..333: mol_type = other DNA
cagtctgccctgactcagcctgcctccgtgtctgggtctcctggacagtcgatcaccatctcctgcactggaaccagcagtgacgttagggctaataactatgtctcctggtaccaacagcacccaggcaaagcccccaaactcatgatttatgagagtagtgcgcggccctcaggggtttctaatcgcttctctggctccaagtctggcaacacggcctccctgaccatctctgggctccaggctgaggacgaggctgattattactgcagctcatatgattggtggttccgccccaaggtgttcggcggagggaccaagctgaccgtccta

SEQ ID NO: 204 - protein, 111 aa, synthetic construct
  REGION 1..111: note = anti-CD47 Kc4B1 kappa variable light domain
QSALTQPASVSGSPGQSITISCTGTSSDVRANNYVSWYQQHPGKAPKLMIYESSARPSGVSNRFSGSKSGNTASLTISGLQAEDEADYYCSSYDWWFRPKVFGGGTKLTVL

SEQ ID NO: 205 - DNA, 333 bp, synthetic construct
  misc_feature 1..333: note = anti-CD47 Kc4E2 kappa variable light domain
  source 1..333: mol_type = other DNA
cagtctgccctgactcagcctgcctccgtgtctgggtctcctggacagtcgatcaccatctcctgcactggaaccagcagtgacgtttattataataagtatgtctcctggtaccaacagcacccaggcaaagcccccaaactcatgatttatgagagtagtaagcggccctcaggggtttctaatcgcttctctggctccaagtctggcaacacggcctccctgaccatctctgggctccaggctgaggacgaggctgattattactgcagctcatatgattggtggttccgccccaaggtgttcggcggagggaccaagctgaccgtccta

SEQ ID NO: 206 - protein, 111 aa, synthetic construct
  REGION 1..111: note = anti-CD47 Kc4E2 kappa variable light domain
QSALTQPASVSGSPGQSITISCTGTSSDVYYNKYVSWYQQHPGKAPKLMIYESSKRPSGVSNRFSGSKSGNTASLTISGLQAEDEADYYCSSYDWWFRPKVFGGGTKLTVL

SEQ ID NO: 207 - DNA, 336 bp, synthetic construct
  misc_feature 1..336: note = anti-CD19 C2 lambda variable light domain
  source 1..336: mol_type = other DNA
aattttatgctgactcagccccactctgtgtcggagtctccggggaagacggtaaccatctcctgcacccgcagcagtggctctatcgaagataagtatgtgcagtggtaccagcagcgcccgggcagttcccccaccattgtgatctattatgataacgaaagaccctctggggtccctgatcggttctctggctccatcgacagctcctccaactctgcctccctcaccatctctggactgaagactgaggacgaggctgactactactgtcagacctacgaccagagcctgtatggttgggtgttcggcggagggaccaagctgaccgtccta

SEQ ID NO: 208 - protein, 112 aa, synthetic construct
  REGION 1..112: note = anti-CD19 C2 lambda variable light domain
NFMLTQPHSVSESPGKTVTISCTRSSGSIEDKYVQWYQQRPGSSPTIVIYYDNERPSGVPDRFSGSIDSSSNSASLTISGLKTEDEADYYCQTYDQSLYGWVFGGGTKLTVL

SEQ ID NO: 209 - DNA, 336 bp, synthetic construct
  misc_feature 1..336: note = anti-CD19 A6 lambda variable light domain
  source 1..336: mol_type = other DNA
aattttatgctgactcagccccactctgtgtcggagtctccggggaagacggtaaccatctcctgcacccgcagcagtggctctatcggtgataagtatgtgcagtggtaccagcagcgcccgggcagttcccccaccattgtgatctattatgataacgaaagaccctctggggtccctgatcggttctctggctccatcgacagctcctccaactctgcctccctcaccatctctggactgaagactgaggacgaggctgactactactgtcagacgtacgacgagagcctgtatggttgggtgttcggcggagggaccaagctgaccgtccta

SEQ ID NO: 210 - protein, 112 aa, synthetic construct
  REGION 1..112: note = anti-CD19 A6 lambda variable light domain
NFMLTQPHSVSESPGKTVTISCTRSSGSIGDKYVQWYQQRPGSSPTIVIYYDNERPSGVPDRFSGSIDSSSNSASLTISGLKTEDEADYYCQTYDESLYGWVFGGGTKLTVL

SEQ ID NO: 211 - DNA, 336 bp, synthetic construct
  misc_feature 1..336: note = anti-CD19 C6 lambda variable light domain
  source 1..336: mol_type = other DNA
aattttatgctgactcagccccactctgtgtcggagtctccggggaagacggtaaccatctcctgcacccgcagcagtggctctatcaatgataagtatgtgcagtggtaccagcagcgcccgggcagttcccccaccattgtgatctattttgataacgaaagaccctctggggtccctgatcggttctctggctccatcgacagctcctccaactctgcctccctcaccatctctggactgaagactgaggacgaggctgactactactgtcagacctacgacaccagcctgtatggttgggtgttcggcggagggaccaagctgaccgtccta

SEQ ID NO: 212 - protein, 112 aa, synthetic construct
  REGION 1..112: note = anti-CD19 C6 lambda variable light domain
NFMLTQPHSVSESPGKTVTISCTRSSGSINDKYVQWYQQRPGSSPTIVIYFDNERPSGVPDRFSGSIDSSSNSASLTISGLKTEDEADYYCQTYDTSLYGWVFGGGTKLTVL

SEQ ID NO: 213 - DNA, 336 bp, synthetic construct
  misc_feature 1..336: note = anti-CD19 C9 lambda variable light domain
  source 1..336: mol_type = other DNA
aattttatgctgactcagccccactctgtgtcggagtctccggggaagacggtaaccatctcctgcacccgcagcagtggctctatcgctgataagtatgtgcagtggtaccagcagcgcccgggcagttcccccaccattgtgatctattatgataacgaaagaccctctggggtccctgatcggttctctggctccatcgacagctcctccaactctgcctccctcaccatctctggactgaagactgaggacgaggctgactactactgtcagacctacgacgagagcctgtatggttgggtgttcggcggagggaccaagctgaccgtccta

SEQ ID NO: 214 - protein, 112 aa, synthetic construct
  REGION 1..112: note = anti-CD19 C9 lambda variable light domain
NFMLTQPHSVSESPGKTVTISCTRSSGSIADKYVQWYQQRPGSSPTIVIYYDNERPSGVPDRFSGSIDSSSNSASLTISGLKTEDEADYYCQTYDESLYGWVFGGGTKLTVL

SEQ ID NO: 215 - DNA, 336 bp, synthetic construct
  misc_feature 1..336: note = anti-CD19 B11 lambda variable light domain
  source 1..336: mol_type = other DNA
aattttatgctgactcagccccactctgtgtcggagtctccggggaagacggtaaccatctcctgcacccgcagcagtggctctatcgaagataagtatgtgcagtggtaccagcagcgcccgggcagttcccccaccattgtgatctattatgataacgaaagaccctctggggtccctgatcggttctctggctccatcgacagctcctccaactctgcctccctcaccatctctggactgaagactgaggacgaggctgactactactgtcagacctacgacaacagcctgtatggttgggtgttcggcggagggaccaagctgaccgtccta

SEQ ID NO: 216 - protein, 112 aa, synthetic construct
  REGION 1..112: note = anti-CD19 B11 lambda variable light domain
NFMLTQPHSVSESPGKTVTISCTRSSGSIEDKYVQWYQQRPGSSPTIVIYYDNERPSGVPDRFSGSIDSSSNSASLTISGLKTEDEADYYCQTYDNSLYGWVFGGGTKLTVL

SEQ ID NO: 217 - DNA, 336 bp, synthetic construct
  misc_feature 1..336: note = anti-CD19 D11 lambda variable light domain
  source 1..336: mol_type = other DNA
aattttatgctgactcagccccactctgtgtcggagtctccggggaagacggtaaccatctcctgcacccgcagcagtggcagcatcgatgataagtttgtgcagtggtaccagcagcgcccgggcagttcccccaccactgtgatctattatgataacattagaccctctggggtccctgatcggttctctggctccatcgacagctcctccaactctgcctccctcaccatctctggactgaagactgaggacgaggctgactactactgtcagtcctatgacgcgagcctgtatggttgggtgttcggcggagggaccaagctgaccgtccta

SEQ ID NO: 218 - protein, 112 aa, synthetic construct
  REGION 1..112: note = anti-CD19 D11 lambda variable light domain
NFMLTQPHSVSESPGKTVTISCTRSSGSIDDKFVQWYQQRPGSSPTTVIYYDNIRPSGVPDRFSGSIDSSSNSASLTISGLKTEDEADYYCQSYDASLYGWVFGGGTKLTVL

SEQ ID NO: 219 - DNA, 336 bp, synthetic construct
  misc_feature 1..336: note = anti-CD19 B7 lambda variable light domain
  source 1..336: mol_type = other DNA
aattttatgctgactcagccccactctgtgtcggagtctccggggaagacggtaaccatctcctgcacccgcagcagtggctctatcgcggataagtatgtgcagtggtaccagcagcgcccgggcagttcccccaccactgtgatctatgaggataaccaaagaccctctggggtccctgatcggttctctggctccatcgacagctcctccaactctgcctccctcaccatctctggactgaagactgaggacgaggctgactactactgtcagtcctatgacagcagcctgtatggttgggtgttcggcggagggaccaagctgaccgtccta

SEQ ID NO: 220 - protein, 112 aa, synthetic construct
  REGION 1..112: note = anti-CD19 B7 lambda variable light domain
NFMLTQPHSVSESPGKTVTISCTRSSGSIADKYVQWYQQRPGSSPTTVIYEDNQRPSGVPDRFSGSIDSSSNSASLTISGLKTEDEADYYCQSYDSSLYGWVFGGGTKLTVL

SEQ ID NO: 221 - DNA, 330 bp, synthetic construct
  misc_feature 1..330: note = dummy variable light domain 1
  source 1..330: mol_type = other DNA
cagtctgtgttgacgcagccgccctcagtgtctgcggccccaggacagaaggtcaccatctcctgctctggaagcagctccaatattgagactggttctgtatcctggtaccagcagctcccaggaacagcccccaaactcctcatttatgacaataataagcgaccctcagggattcctgaccgattctctggctccaagtctggcacgtcagccaccctgggcatcaccggactccagactggggacgaggccgattattactgcggaacatgggatgacagcctgcctggatgggtgttcggcggagggaccaagctgaccgtccta

SEQ ID NO: 222 - protein, 110 aa, synthetic construct
  REGION 1..110: note = dummy variable light domain 1
QSVLTQPPSVSAAPGQKVTISCSGSSSNIETGSVSWYQQLPGTAPKLLIYDNNKRPSGIPDRFSGSKSGTSATLGITGLQTGDEADYYCGTWDDSLPGWVFGGGTKLTVL

SEQ ID NO: 223 - DNA, 333 bp, synthetic construct
  misc_feature 1..333: note = dummy variable light domain 2
  source 1..333: mol_type = other DNA
gaaatagtgatgacgcagtctccagccaccctgtctgtgtctccaggggaaagagccaccctctcctgcagggccagtcagacggttaagaataatttagcctggtaccagcagaaacctggccaggctcccaggctcctcatctatggtgcatccaccagggccactggtatcccagccaggttcagtggcagtgggtctgggacagagttcactctcaccatcagcagcctgcagtctgaagattttgcagtttattactgtcagcagtataacaactggttgcccatcaacccctataccttcggccaagggaccaaggtggaaatcaaa

SEQ ID NO: 224 - protein, 111 aa, synthetic construct
  REGION 1..111: note = dummy variable light domain 2
EIVMTQSPATLSVSPGERATLSCRASQTVKNNLAWYQQKPGQAPRLLIYGASTRATGIPARFSGSGSGTEFTLTISSLQSEDFAVYYCQQYNNWLPINPYTFGQGTKVEIK

SEQ ID NO: 225 - protein, 8 aa, synthetic construct
  REGION 1..8: note = anti-CD47 heavy chain CDHR1
GFTFSSYA

SEQ ID NO: 226 - protein, 8 aa, synthetic construct
  REGION 1..8: note = anti-CD47 heavy chain CDHR2
ISGSGGST

SEQ ID NO: 227 - protein, 9 aa, synthetic construct
  REGION 1..9: note = anti-CD47 heavy chain CDHR3
AKSYGAFDY

SEQ ID NO: 228 - protein, 6 aa, synthetic construct
  REGION 1..6: note = anti-CD47 kappa light chain CDRL1
QDINKY

SEQ ID NO: 229 - protein, 6 aa, synthetic construct
  REGION 1..6: note = anti-CD47 kappa light chain CDRL1
QDINRY

SEQ ID NO: 230 - protein, 6 aa, synthetic construct
  REGION 1..6: note = anti-CD47 kappa light chain CDRL1
QNIGKY

SEQ ID NO: 231 - protein, 6 aa, synthetic construct
  REGION 1..6: note = anti-CD47 kappa light chain CDRL1
QSIARY

SEQ ID NO: 232 - protein, 6 aa, synthetic construct
  REGION 1..6: note = anti-CD47 kappa light chain CDRL1
QSIASY

SEQ ID NO: 233 - protein, 6 aa, synthetic construct
  REGION 1..6: note = anti-CD47 kappa light chain CDRL1
QSIDKY

SEQ ID NO: 234 - protein, 6 aa, synthetic construct
  REGION 1..6: note = anti-CD47 kappa light chain CDRL1
QSIDRY

SEQ ID NO: 235 - protein, 6 aa, synthetic construct
  REGION 1..6: note = anti-CD47 kappa light chain CDRL1
QSIGKY

SEQ ID NO: 236 - protein, 6 aa, synthetic construct
  REGION 1..6: note = anti-CD47 kappa light chain CDRL1
QSIGRY

SEQ ID NO: 237 - protein, 6 aa, synthetic construct
  REGION 1..6: note = anti-CD47 kappa light chain CDRL1
QSINRY

SEQ ID NO: 238 - protein, 6 aa, synthetic construct
  REGION 1..6: note = anti-CD47 kappa light chain CDRL1
QSISKY

SEQ ID NO: 239 - protein, 6 aa, synthetic construct
  REGION 1..6: note = anti-CD47 kappa light chain CDRL1
QSISRY

SEQ ID NO: 240 - protein, 6 aa, synthetic construct
  REGION 1..6: note = anti-CD47 kappa light chain CDRL1
QSISSY

SEQ ID NO: 241 - protein, 6 aa, synthetic construct
  REGION 1..6: note = anti-CD47 kappa light chain CDRL1
QSIAKY

SEQ ID NO: 242-245 - skipped (4 entries)

SEQ ID NO: 246 - protein, 10 aa, synthetic construct
  REGION 1..10: note = anti-CD47 kappa light chain CDRL3
QQKHPRGPRT

SEQ ID NO: 247 - protein, 10 aa, synthetic construct
  REGION 1..10: note = anti-CD47 kappa light chain CDRL3
QQFHKRAPQT

SEQ ID NO: 248 - protein, 10 aa, synthetic construct
  REGION 1..10: note = anti-CD47 kappa light chain CDRL3
QQFHKRRPQT

SEQ ID NO: 249 - protein, 10 aa, synthetic construct
  REGION 1..10: note = anti-CD47 kappa light chain CDRL3
QQFHKRSPQT

SEQ ID NO: 250 - protein, 10 aa, synthetic construct
  REGION 1..10: note = anti-CD47 kappa light chain CDRL3
QQKHPRAPRT

SEQ ID NO: 251 - protein, 10 aa, synthetic construct
  REGION 1..10: note = anti-CD47 kappa light chain CDRL3
QQKHPRSPRT

SEQ ID NO: 252 - protein, 10 aa, synthetic construct
  REGION 1..10: note = anti-CD47 kappa light chain CDRL3
QQKHPRYPRT

SEQ ID NO: 253 - protein, 10 aa, synthetic construct
  REGION 1..10: note = anti-CD47 kappa light chain CDRL3
QQKHPRNPRT

SEQ ID NO: 254 - protein, 10 aa, synthetic construct
  REGION 1..10: note = anti-CD47 kappa light chain CDRL3
QQMHPRAPKT

SEQ ID NO: 255 - protein, 10 aa, synthetic construct
  REGION 1..10: note = anti-CD47 kappa light chain CDRL3
QQMHPRGPKT

SEQ ID NO: 256 - protein, 10 aa, synthetic construct
  REGION 1..10: note = anti-CD47 kappa light chain CDRL3
QQMHPRSPKT

SEQ ID NO: 257 - protein, 10 aa, synthetic construct
  REGION 1..10: note = anti-CD47 kappa light chain CDRL3
QQRHPRAPRT

SEQ ID NO: 258 - protein, 10 aa, synthetic construct
  REGION 1..10: note = anti-CD47 kappa light chain CDRL3
QQRHKRSPQT

SEQ ID NO: 259 - protein, 10 aa, synthetic construct
  REGION 1..10: note = anti-CD47 kappa light chain CDRL3
QQRHPRGPRT

SEQ ID NO: 260 - protein, 10 aa, synthetic construct
  REGION 1..10: note = anti-CD47 kappa light chain CDRL3
QQRHPRGPST

SEQ ID NO: 261 - protein, 10 aa, synthetic construct
  REGION 1..10: note = anti-CD47 kappa light chain CDRL3
QQRHPRGPTT

SEQ ID NO: 262 - protein, 9 aa, synthetic construct
  REGION 1..9: note = anti-CD47 lambda light chain CDRL1
SSDVGGYNY

SEQ ID NO: 263 - protein, 9 aa, synthetic construct
  REGION 1..9: note = anti-CD47 lambda light chain CDRL1
SSDVERKNY

SEQ ID NO: 264 - protein, 9 aa, synthetic construct
  REGION 1..9: note = anti-CD47 lambda light chain CDRL1
SSDVRANNY

SEQ ID NO: 265 - protein, 9 aa, synthetic construct
  REGION 1..9: note = anti-CD47 lambda light chain CDRL1
SSDVYYNKY

SEQ ID NO: 266 - protein, 9 aa, synthetic construct
  REGION 1..9: note = anti-CD47 lambda light chain CDRL1
SSDVGKANY

SEQ ID NO: 267 - protein, 9 aa, synthetic construct
  REGION 1..9: note = anti-CD47 lambda light chain CDRL1
SSDVRGNNY

SEQ ID NO: 268 - protein, 9 aa, synthetic construct
  REGION 1..9: note = anti-CD47 lambda light chain CDRL1
SSDVSARNY

SEQ ID NO: 269 - protein, 9 aa, synthetic construct
  REGION 1..9: note = anti-CD47 lambda light chain CDRL1
SSDVNSANY

SEQ ID NO: 270 - protein, 9 aa, synthetic construct
  REGION 1..9: note = anti-CD47 lambda light chain CDRL1
SSDVRAANY

SEQ ID NO: 271 - protein, 9 aa, synthetic construct
  REGION 1..9: note = anti-CD47 lambda light chain CDRL1
SSDVRRANY

SEQ ID NO: 272 - protein, 9 aa, synthetic construct
  REGION 1..9: note = anti-CD47 lambda light chain CDRL1
SSDVNNTNY

SEQ ID NO: 273-280 - skipped (8 entries)

SEQ ID NO: 281 - protein, 11 aa, synthetic construct
  REGION 1..11: note = anti-CD47 lambda light chain CDRL3
SSYDWWFRPKV

SEQ ID NO: 282 - protein, 94 aa, Homo sapiens
DIQMTQSPSSLSASVGDRVTITCQASQDISNYLNWYQQKPGKAPKLLIYDASNLETGVPSRFSGSGSGTDFTFTISSLQPEDIATYYCQYDNLP

SEQ ID NO: 283 - DNA, 21 bp, synthetic construct
  misc_feature 1..21: note = pNDS1 mycseq primer
  source 1..21: mol_type = other DNA
ctcttctgagatgagtttttg

SEQ ID NO: 284 - DNA, 30 bp, synthetic construct
  misc_feature 1..30: note = pNDS1 gene3leader primer
  source 1..30: mol_type = other DNA
ttattattcgcaattcctttagttgttcct

SEQ ID NO: 285 - protein, 110 aa, synthetic construct
  REGION 1..110: note = 5A3-VL
DIQMTQSPSSLSASVGDRVTITCQASQDINKYLNWYQQKPGKAPKLLIYGASRLETGVPSRFSGSGSGTDFTFTISSLQPEDIATYYCQQKHPRGPRTFGQGTKVEIKRT

SEQ ID NO: 286 - protein, 110 aa, synthetic construct
  REGION 1..110: note = 5A3-M3-VL
DIQMTQSPSSLSASVGDRVTITCQASQSISSYLNWYQQKPGKAPKLLIYAASSLETGVPSRFSGSGSGTDFTFTISSLQPEDIATYYCQQKHPRGPRTFGQGTKVEIKRT

SEQ ID NO: 287 - protein, 110 aa, synthetic construct
  REGION 1..110: note = 5A3-M5-VL
DIQMTQSPSSLSASVGDRVTITCQASQDINKYLNWYQQKPGKAPKLLIYGASRLETGVPSRFSGSGSGTDFTFTISSLQPEDIATYYCQQKHPRYPRTFGQGTKVEIKRT